European Patent Specification EP 3 526 256 B1, published September 10, 2025. Title: ANTI-LAG-3 ANTIBODIES AND METHODS OF USE THEREOF. Applicant: AGENUS INC. The sequence listing filed with the application follows.

SEQUENCE LISTING (228 sequences)

SEQ ID NO: 1 - protein, 120 aa, Artificial Sequence
  source: /note="Description of Artificial Sequence: Synthetic polypeptide"
QVQLKQSGAELVKPGASVKLSCTASGFNIKDTYMYWVKQRPEQGLEWIGRIDPANGNTKYDPKLQGKATITADTSSNTVYLQLSSLTSEDTAVFYCVIYSYRYDVGGFDYWGQGTTLTVS

SEQ ID NO: 2 - protein, 108 aa, Artificial Sequence
  source: /note="Description of Artificial Sequence: Synthetic polypeptide"
EIVLTQSPALMAASPGEKVTITCSVSSSISSSNLHWYQQKSGTSPKLWIYGTSNLASGVPVRFSGSGSGTSYSLTISSMEAEDAATYYCQQWSSYPFTFGSGTKLEIK

SEQ ID NO: 3 - protein, 120 aa, Artificial Sequence
  source: /note="Description of Artificial Sequence: Synthetic polypeptide"
DVQLVESGAELVKPGASVKLSCTASGFTIKDTYIHWVKQRPEQGLEWIGEIDPANGNTKYDPKFQGKATITADTSSNTAYLQLSSLTSEDTAVYYCATYYYRYDVGGFDYWGQGTTLTVS

SEQ ID NO: 4 - protein, 108 aa, Artificial Sequence
  source: /note="Description of Artificial Sequence: Synthetic polypeptide"
DIVLTQSPALMAASPGEKVTITCSVSSSISSSNLHWFQQKSGTSPKLWIYGTSNLASGVPVRFSGSGSGTSYSLTISNMEAEDAATYYCQQWNSYPLTFGAGTKLELK

SEQ ID NO: 5 - protein, 120 aa, Artificial Sequence
  source: /note="Description of Artificial Sequence: Synthetic polypeptide"
EVQLQQSGAELVKPGASVKLSCTASGFNIKDTYMYWVKQRPEQGLDWIGRIDPANGNTKFDPKFQGKATITADTSSNTAYLQLSSLTSEDTAVYYCSTYYYRYDVGGFDYWGQGTTLTVS

SEQ ID NO: 6 - protein, 108 aa, Artificial Sequence
  source: /note="Description of Artificial Sequence: Synthetic polypeptide"
DIVLTQSPALMAASPGEKVTITCSVSSSISSSNLHWYQQKSGTSPKLWIYGTSNLASGVPVRFSGSGSGTSYSLTISSMEAEDAATYYCQQWSSYPFTFGSGTKLEIK

SEQ ID NO: 7 - protein, 120 aa, Artificial Sequence
  source: /note="Description of Artificial Sequence: Synthetic polypeptide"
EVQLQQSGAELVKPGASVKLSCTASGFNIKDTYIYWVKQRPERGLEWIGRIDPANGNTKFDPKFQGTATITADTSSNTAYLQLSSLTSEDTAVYYCTTYFYRYDVGGFDYWGQGTTLTVS

SEQ ID NO: 8 - protein, 108 aa, Artificial Sequence
  source: /note="Description of Artificial Sequence: Synthetic polypeptide"
ENVLTQSPALMAASPGEKVTITCSVSSSISSSNLHWYQQKSGTSPKLWIYGTSNLASGVPVRFSGSGSGTSYSLTISSMEAEDAATYYCQQWSSYPFTFGSGTKLEIK

SEQ ID NO: 9 - protein, 120 aa, Artificial Sequence
  source: /note="Description of Artificial Sequence: Synthetic polypeptide"
QVQLQQSGAELVKPGASVELSCTASGFNIRDTYMYWVKQRPEQGLEWIGRIDPANGNTKFDPKFQDRATMTADTSSNTAYLQLSSLTSEDTAVYYCTTYFYRYDVGGFDYWGQGTTLTVS

SEQ ID NO: 10 - protein, 108 aa, Artificial Sequence
  source: /note="Description of Artificial Sequence: Synthetic polypeptide"
ENVLTQSPALMAASPGEKVTITCSVSSSISSSNLHWFQQKSGTSPKLWIYGTSNLASGVPVRFSGSGSGTSYSLTISSMEAEDAATYYCQQWSSYPFTFGSGTKLEIK

SEQ ID NO: 11 - protein, 120 aa, Artificial Sequence
  source: /note="Description of Artificial Sequence: Synthetic polypeptide"
QVQLKQSGAELVKPGASVKLSCTASGFNIKDNYIHWVKQRPEQGLEWIGSIDPANGNTKYDPKFQGKASITADTSSNTAYLQLSSLTSEDTAVYYCASYFYRYDVGGFDYWGQGTTLTVS

SEQ ID NO: 12 - protein, 108 aa, Artificial Sequence
  source: /note="Description of Artificial Sequence: Synthetic polypeptide"
DVVMTQTPALMAASPGEKVTITCSVSSSISSSNLHWFQQKSGTSPKLWIYGTSNLASGVPVRFSGSGSGTSYSLTISSMEAEDAATYYCQQWSSYPFTFGSGTKLEIK

SEQ ID NO: 13 - protein, 120 aa, Artificial Sequence
  source: /note="Description of Artificial Sequence: Synthetic polypeptide"
QVQLQQPGAELVKPGASVKLSCTVSGFNIKDTYIHWVKQRPEQGLEWIGEIDPANGNSKYAPRFQGKATITADTSSNTAYLQLSSLTSEDTAVYYCATYYYRYDVGGFDYWGQGTTLTVS

SEQ ID NO: 14 - protein, 120 aa, Artificial Sequence
  source: /note="Description of Artificial Sequence: Synthetic polypeptide"
QVQLQQPGAELVKPGASVKLSCTASGFNIKDTYIHWVKQRPEQGLDWVGEIDPANGHTKYDPKFQGKATITADTSSNTAYLQLSSLTSEDTAVYYCATYYYRYDVGGFDYWGQGTTLTVS

SEQ ID NO: 15 - protein, 120 aa, Artificial Sequence
  source: /note="Description of Artificial Sequence: Synthetic polypeptide"
QVQMKQSGAELVKPGASVKLSCTASGFNIKDTYIHWVKQRPEQGLEWIGEIDPANDNTKYDPKFQGKATITADTSSNTAYLQLSSLTSEDTAVYYCATYYYRYDVGGFDYWGQGTTLTVS

SEQ ID NO: 16 - protein, 108 aa, Artificial Sequence
  source: /note="Description of Artificial Sequence: Synthetic polypeptide"
EILLTQSPALMAASPGEKVTITCSVSSSISSSNLHWFQQKSGTSPKLWIYGTSNLASGVPVRFSGSGSGTSYSLTISSMEAEDAATYYCQQWSSYPFTFGSGTKLEIK

SEQ ID NO: 17 - protein, 120 aa, Artificial Sequence
  source: /note="Description of Artificial Sequence: Synthetic polypeptide"
QVQLKQSGAELVKPGASVKLSCTASGFNIKDTYMYWVKQRPEQGLEWIGRIDPANGNTKYDPKFQGKATITADTSSNTVYLQLSSLTSEDTAVFYCVIYSYRYDVGGFDYWGQGTTLTVS

SEQ ID NO: 18 - protein, 108 aa, Artificial Sequence
  source: /note="Description of Artificial Sequence: Synthetic polypeptide"
ENVLTQSPALMAASPGEKVTITCSVSSSISSSNLHWYQQKSGTSPKLWIYGTSNLASGVPVRFSGSGSGTSYSLTISSMEAEDAATYYCQQWSSYPHTFGGGTKLEIK

SEQ ID NO: 19 - protein, 120 aa, Artificial Sequence
  source: /note="Description of Artificial Sequence: Synthetic polypeptide"
QVQLQQPGAELVKPGASVKLSCTASGFNIKDTYMYWVKQRPEQGLDWIGRIDPANGNTHFDPKFQGKATITADTSSNTAYLQLSSLTSEDTAVYYCSTYFYRYDVGGFDYWGQGTTLTVS

SEQ ID NO: 20 - protein, 120 aa, Artificial Sequence
  source: /note="Description of Artificial Sequence: Synthetic polypeptide"
QVQLQQPGAELVKPGASVELSCTASGFNIRDTYMYWVKQRPEQGLEWIGRIDPANGNTKFDPKFQDRATMTADTSSNTAYLQLSSLTSEDTAVYYCTTYFYRYDVGGFDYWGQGTTLTVS

SEQ ID NO: 21 - protein, 108 aa, Artificial Sequence
  source: /note="Description of Artificial Sequence: Synthetic polypeptide"
DIVLTQSPALMAASPGEKVTITCSVSSSISSSNLHWFQQKSGTSPKLWIYGTSNLASGVPVRFSGSGSGTSYSLTISSMEAEDAATYYCQQWSSYPFTFGSGTKLEIK

SEQ ID NO: 22 - protein, 120 aa, Artificial Sequence
  source: /note="Description of Artificial Sequence: Synthetic polypeptide"
QVQLKQSGAELVKPGASVELSCTASGFNIRDTYMYWVKQRPEQGLEWIGRIDPANGNTKFDPKFQDRATMTADTSSNTAYLQLSSLTSEDTAVYYCTTYFYRYDVGGFDYWGQGTTLTVS

SEQ ID NO: 23 - protein, 108 aa, Artificial Sequence
  source: /note="Description of Artificial Sequence: Synthetic polypeptide"
ENVLTQSPALMAASPGEKVTITCSVSSSISSSTLHWFQQKSGTSPKLWIYGTSNLASGVPVRFSGSGSGTSYSLTISSMEAEDAATYYCQQWSSYPWTFGGGTKLEIK

SEQ ID NO: 24 - protein, 120 aa, Artificial Sequence
  source: /note="Description of Artificial Sequence: Synthetic polypeptide"
EVQLQQSGAELVKPGASVKLSCTASGFNIKDTYIHWVKQRPEQGLEWIGEIDPANGNTKYDPKFQGKATITADTSSNTAYLQLSSLTSEDTAVYYCATYYYRYDVGGFDYWGQGTTLTVS

SEQ ID NO: 25 - protein, 108 aa, Artificial Sequence
  source: /note="Description of Artificial Sequence: Synthetic polypeptide"
DVVMTQTPALMAASPGEKVTITCSVSSSISSSNLHWYQQKSGTSPKLWIYGTSNLASGVPVRFSGSGSGTSYSLTISSMEAEDAATYYCQQWSSYPFTFGSGTKLEIK

SEQ ID NO: 26 - protein, 108 aa, Artificial Sequence
  source: /note="Description of Artificial Sequence: Synthetic polypeptide"
ENVLTQSPALMAASPGEKVTITCSVSSSISSSNLHWYQQKSGTSPKLWIYGTSNLASGVPVRFSGSGSGTSYSLTISSMEAEDAATYYCQQWSSYPLTFGAGTKLELK

SEQ ID NO: 27 - protein, 120 aa, Artificial Sequence
  source: /note="Description of Artificial Sequence: Synthetic polypeptide"
QVQLQQPGAELVKPGASVELSCTASGFNIRDTYMYWVKQRPEQGLEWIGRIDPANGNTKFDPKFQDRATMTADTSSNTAYLQLSSLTSADTAVYYCTTYFYRYDVGGFDYWGQGTTLTVS

SEQ ID NO: 28 - protein, 108 aa, Artificial Sequence
  source: /note="Description of Artificial Sequence: Synthetic polypeptide"
DIVLTQSPALMAASPGEKVTITCSVSSSISSSNLHWYQQKSGTSPKLWIYGTSNLASGVPVRFSGSGSGTSYSLTISNMEAEDAATYYCQQWSSYPFTFGSGTKLEIK

SEQ ID NO: 29 - protein, 120 aa, Artificial Sequence
  source: /note="Description of Artificial Sequence: Synthetic polypeptide"
QVQLQQPGAELVKPGASVKLSCTASGFNIKDNYIHWVKQRPEQGLEWIGSIDPANGNTKYDPKFQGKASITADTSSNTAYLQLSSLTSEDTAVYYCASYFYRYDVGGFDYWGQGTTLTVS

SEQ ID NO: 30 - protein, 108 aa, Artificial Sequence
  source: /note="Description of Artificial Sequence: Synthetic polypeptide"
EIVLTQSPALMAASPGEKVTITCSVSSSISSSNLHWYQQKSGTSPKLWIYGTSNLASGVPVRFSGSGSGTSYSLTISSMEAEDAATYYCQQWSSYPHTFGGGTKLEIK

SEQ ID NO: 31 - protein, 120 aa, Artificial Sequence
  source: /note="Description of Artificial Sequence: Synthetic polypeptide"
QVQLQQSGAELVKPGASVKLSCTASGFNIKDNYIHWVKQRPEQGLEWIGSIDPANGNTKYDPKFQGKASITADTSSNTAYLQLSSLTSEGTAVYYCASYFYRYDVGGFDYWGQGTTLTVS

SEQ ID NO: 32 - protein, 108 aa, Artificial Sequence
  source: /note="Description of Artificial Sequence: Synthetic polypeptide"
EIVLTQSPALMAASPGEKVTITCSVSSSISSSNLHWFQQKSGTSPKLWIYGTSNLASGVPVRFSGSGSGTSYSLTISSMEAEDAATYYCQQWSSYPFTFGSGTKLEIK

SEQ ID NO: 33 - protein, 120 aa, Artificial Sequence
  source: /note="Description of Artificial Sequence: Synthetic polypeptide"
EVQLQQSGAELVKPGASVELSCTASGFNIRDTYMYWVKQRPEQGLEWIGRIDPANGNTKFDPKFQDRATMTADTSSNTAYLQLSSLTSEDTAVYYCTTYFYRYDVGGFDYWGQGTTLTVS

SEQ ID NO: 34 - protein, 108 aa, Artificial Sequence
  source: /note="Description of Artificial Sequence: Synthetic polypeptide"
QIVLTQSPALMAASPGEKVTITCSVSSSISSSNLHWYQQKSGTSPKLWIYGTSNLASGVPVRFSGSGSGTSYSLTISSMEAEDAATYYCQQWSSYPFTFGSGTKLEIK

SEQ ID NO: 35 - protein, 120 aa, Artificial Sequence
  source: /note="Description of Artificial Sequence: Synthetic polypeptide"
QVQLQQPGAELVKPGASVKLSCTASGFNIKDTYIHWVKQRPEQGLEWIGEIDPANDNTKYDPKFQGKATITADTSSNTAYLQLSSLTSEDTAVYYCATYYYRYDVGGFDYWGQGTTLTVS

SEQ ID NO: 36 - protein, 120 aa, Artificial Sequence
  source: /note="Description of Artificial Sequence: Synthetic polypeptide"
QVQLQQSGAELVKPGASVKLSCTASGFNIKDNYMDWVKQRPEQGLEWIGKIDPANGNTKYDPKFQGKATITADTSSNTAYLQLSSLTSEDTAVYYCATYYYRYDVGGFDYWGQGTTLTVS

SEQ ID NO: 37 - protein, 108 aa, Artificial Sequence
  source: /note="Description of Artificial Sequence: Synthetic polypeptide"
DIVLTQSPALMAASPGEKVTITCSVSSSISSSNLHWFQQKSGTPPKLWIYGTSNLASGVPVRFSGSGSGTSYSLTISSMEAEDAATYYCQQWSSYPFTFGSGTKLEIK

SEQ ID NO: 38 - protein, 120 aa, Artificial Sequence
  source: /note="Description of Artificial Sequence: Synthetic polypeptide"
QVQLKESGAELVKPGASVELSCTASGFNIRDTYMYWVKQRPEQGLEWIGRIDPANGNTKFDPKFQDRATMTADTSSNTAYLQLSSLTSEDTAVYYCTTYFYRYDVGGFDYWGQGTTLTVS

SEQ ID NO: 39 - protein, 120 aa, Artificial Sequence
  source: /note="Description of Artificial Sequence: Synthetic polypeptide"
QVQMKQSGAELVKPGASVKLSCTASGFNIKDTYIHWVKQRPGQGLEWIGEIDPANGNTKYDPKFQGKATITADTSSNTAYLQLSSLTSEDTAVYYCATYYYRYDVGGFDYWGQGTTLTVS

SEQ ID NO: 40 - protein, 108 aa, Artificial Sequence
  source: /note="Description of Artificial Sequence: Synthetic polypeptide"
DIVLTQSPALMAASPGEKVTITCSVSSSISSSNLYWFQQKSGTSPKLWIYGTSNLASGVPVRFSGSGSGTSYSLTISSMEAEDAATYYCQQWSSYPFTFGSGTKLEIK

SEQ ID NO: 41 - protein, 108 aa, Artificial Sequence
  source: /note="Description of Artificial Sequence: Synthetic polypeptide"
EILLTQSPALMAASPGEKVTITCSVSSSISSSNLHWYQQKSGTSPKLWIYGTSNLASGVPVRFSGSGSGTSYSLTISSMEAEDAATYYCQQWSSYPFTFGSGTKLEIK

SEQ ID NO: 42 - protein, 120 aa, Artificial Sequence
  source: /note="Description of Artificial Sequence: Synthetic polypeptide"
QVQLQQPGAELVKPGASVKLSCTASGFNIKDNYMDWVKQRPEQGLEWIGKIDPANGNTKYDPKFQGKATITADTSSNTAYLQLSSLTSEDTAVYYCATYYYRYDVGGFDYWGQGTTLTVS

SEQ ID NO: 43 - protein, 108 aa, Artificial Sequence
  source: /note="Description of Artificial Sequence: Synthetic polypeptide"
QIVLTQSPALMAASPGEKVTITCSVSSSISSSNLHWFQQKSGTSPKLWIYGTSNLASGVPVRFSGSGSGTSYSLTISSMEAEDAATYYCQQWSSYPFTFGSGTKLEIK

SEQ ID NO: 44 - protein, 108 aa, Artificial Sequence
  source: /note="Description of Artificial Sequence: Synthetic polypeptide"
ENVLTQSPALMAASPGEKVTITCSVSSSISSSNLHWYQQKSGTSPKLWIYGTSNLASGVPVRFSGSGSGTSYSLTISSMEAEDAATYYCQQWSTYPFTFGSGTKLEIK

SEQ ID NO: 45 - protein, 120 aa, Artificial Sequence
  source: /note="Description of Artificial Sequence: Synthetic polypeptide"
QVQMKQSGAELVKPGASVKLSCTASGFNIKDNYIHWVKQRPEQGLEWIGSIDPANGNTKYDPKFQGKASITADTSSNTAYLQLSSLTSEDTAVYYCASYFYRYDVGGFDYWGQGTTLTVS

SEQ ID NO: 46 - protein, 120 aa, Artificial Sequence
  source: /note="Description of Artificial Sequence: Synthetic polypeptide"
QVQLQQPGAELVKPGASVELSCTASGFNIRDTYMYWVKQRPEQGLGWIGRIDPANGNTKFDPKFQDRATMTADTSSNTAYLQLSSLTSEDTAVYYCTTYFYRYDVGGFDYWGQGTTLTVS

SEQ ID NO: 47 - protein, 108 aa, Artificial Sequence
  source: /note="Description of Artificial Sequence: Synthetic polypeptide"
EIVLTQSPALMAASPGEKVTITCSVSSSISSSNLHWFRQKSGTSPKLWIYGTSNLASGVPVRFSGSGSGTSYSLTISSMEAEDAATYYCQQWSSYPFTFGSGTKLEIK

SEQ ID NO: 48 - protein, 120 aa, Artificial Sequence
  source: /note="Description of Artificial Sequence: Synthetic polypeptide"
EVKLMESGAELVKPGASAELSCTASGFNIRDTYMYWVKQRPEQGLEWIGRIDPANGNTKFDPKFQDRATMTADTSSNTAYLQLSSLTSEDTAVYYCTTYFYRYDVGGFDYWGQGTTLTVS

SEQ ID NO: 49 - protein, 108 aa, Artificial Sequence
  source: /note="Description of Artificial Sequence: Synthetic polypeptide"
ENVLTQSPALMAASPGEKVTITCSVSSGISSSNLHWYQQKSGTSPKLWIYGTSNLASGVPVRFSGSGSGTSYSLTISSMEAEDAATYYCQQWSRYPWTFGGGTKLEIK

SEQ ID NO: 50 - protein, 108 aa, Artificial Sequence
  source: /note="Description of Artificial Sequence: Synthetic polypeptide"
EIVLTQSPALMAASPGEKVTITCSVSSSISSSNLHWYQQKSGTSPKLWIYGTSNLASGVPVRFSGSGSGTSYSLTISSMEAEDAATYYCQQWSSYPLTFGAGTKLELK

SEQ ID NO: 51 - protein, 120 aa, Artificial Sequence
  source: /note="Description of Artificial Sequence: Synthetic polypeptide"
EVQLQQSGAELVKPGASVKLSCTASGFNIKDTYMYWVKQRPEQGLDWIGRIDPANGNTHFDPKFQGKATITADTSSNTAYLQLSSLTSEDTAVYYCSTYFYRYDVGGFDYWGQGTTLTVS

SEQ ID NO: 52 - protein, 108 aa, Artificial Sequence
  source: /note="Description of Artificial Sequence: Synthetic polypeptide"
QILLTQSPALMAASPGEKVTITCSVSSSISSSNLHWYQQKSGTSPKLWIYGTSNLASGVPVRFSGSGSGTSYSLTISSMEAEDAATYYCQQWSSYPLTFGAGTKLELK

SEQ ID NO: 53 - protein, 120 aa, Artificial Sequence
  source: /note="Description of Artificial Sequence: Synthetic polypeptide"
QVQLQQPGAELVKPGASVKLSCTASGFNIKDNYIHWVKQRPEQGLEWIGSIDPANGNTKYDPKFQGKASITADTSSNTAYLQLSSLTSEDTTVYYCASYFYRYDVGGFDYWGQGTTLTVS

SEQ ID NO: 54 - protein, 120 aa, Artificial Sequence
  source: /note="Description of Artificial Sequence: Synthetic polypeptide"
QVQMKQSGAELVKPGASVELSCTASGFNITDTYMYWVKQRPEQGLEWIGRIDPANGNTKFDPKFQDRATMTADTSSNTAYLQLSSLTSEDTAVYYCTTYFDKYDVGGCDYWGQGTTLTVS

SEQ ID NO: 55 - protein, 108 aa, Artificial Sequence
  source: /note="Description of Artificial Sequence: Synthetic polypeptide"
EIVLTQSPALMAASPGEKVTITCSVSSSISSSNLYWFQHKSGTSPKLWIYGTSNLASGVPVRFSGSGSGTSYSLTISSMDAENAATYYCQQWRSYPFTFGSGTKLEIK

SEQ ID NO: 56 - protein, 121 aa, Artificial Sequence
  source: /note="Description of Artificial Sequence: Synthetic polypeptide"
QVQLVQSGAEVKKPGASVKVSCKASGFNIKDTYIHWVRQAPGQGLEWMGEIDPANDNTKYDPKFQGRVTMTRDTSTSTVYMELSSLRSEDTAVYYCARYYYRYDVGGFDYWGQGTLVTVSS

SEQ ID NO: 57 - protein, 121 aa, Artificial Sequence
  source: /note="Description of Artificial Sequence: Synthetic polypeptide"
QVQLVQSGAEVKKPGASVKVSCKASGFNIKDTYIHWVRQAPGQGLEWMGEIDPANDNTKYDPKFQGRVTITADTSTSTVYMELSSLRSEDTAVYYCATYYYRYDVGGFDYWGQGTLVTVSS

SEQ ID NO: 58 - protein, 121 aa, Artificial Sequence
  source: /note="Description of Artificial Sequence: Synthetic polypeptide"
QVQLVQSGAEVKKPGASVKVSCKASGFNIKDTYIHWVRQAPGQGLEWMGEIDPANDNTKYDPKFQGRVTITADTSSNTVYMELSSLRSEDTAVYYCATYYYRYDVGGFDYWGQGTLVTVSS

SEQ ID NO: 59 - protein, 121 aa, Artificial Sequence
  source: /note="Description of Artificial Sequence: Synthetic polypeptide"
QVQMKQSGAEVKKPGASVKVSCTASGFNIKDTYIHWVRQAPGQGLEWMGEIDPANDNTKYDPKFQGRVTITADTSSNTVYMELSSLRSEDTAVYYCATYYYRYDVGGFDYWGQGTLVTVSS

SEQ ID NO: 60 - protein, 121 aa, Artificial Sequence
  source: /note="Description of Artificial Sequence: Synthetic polypeptide"
QVQMKQSGAEVVKPGASVKVSCTASGFNIKDTYIHWVRQAPGQGLEWIGEIDPANDNTKYDPKFQGRVTITADTSSNTVYLQLSSLRSEDTAVYYCATYYYRYDVGGFDYWGQGTLVTVSS

SEQ ID NO: 61 - protein, 121 aa, Artificial Sequence
  source: /note="Description of Artificial Sequence: Synthetic polypeptide"
QVQMKQSGAEVVKPGASVKVSCTASGFNIKDTYIHWVRQAPGQGLEWIGEIDPANDNTKYDPKFQGRVTITADTSSNTVYLQLSSLRSEDTAVYYCATYYYKYDVGGFDYWGQGTLVTVSS

SEQ ID NO: 62 - protein, 121 aa, Artificial Sequence
  source: /note="Description of Artificial Sequence: Synthetic polypeptide"
QVQMKQSGAEVVKPGASVKVSCTASGFNIKDTYIHWVRQAPGQGLEWIGEIDPANDNTKYDPKFQGRVTITADTSSNTVYLQLSSLRSEDTAVYYCATYYYRYEVGGFDYWGQGTLVTVSS

SEQ ID NO: 63 - protein, 121 aa, Artificial Sequence
  source: /note="Description of Artificial Sequence: Synthetic polypeptide"
QVQLVQSGAEVKKPGASVKVSCKASGFNIKDTYIHWVRQAPGQGLEWMGEIDPANDNTKYDPKFQGRVTITADTSTSTVYMELSSLRSEDTAVYYCATYYYKYDVGGFDYWGQGTLVTVSS

SEQ ID NO: 64 - protein, 121 aa, Artificial Sequence
  source: /note="Description of Artificial Sequence: Synthetic polypeptide"
QVQLVQSGAEVKKPGASVKVSCTASGFNIKDTYIHWVRQAPGQGLEWMGEIDPANDNTKYDPKFQGRVTITADTSTSTVYMELSSLRSEDTAVYYCATYYYKYDVGGFDYWGQGTLVTVSS

SEQ ID NO: 65 - protein, 121 aa, Artificial Sequence
  source: /note="Description of Artificial Sequence: Synthetic polypeptide"
QVQMVQSGAEVKKPGASVKVSCKASGFNIKDTYIHWVRQAPGQGLEWMGEIDPANDNTKYDPKFQGRVTITADTSTSTVYMELSSLRSEDTAVYYCATYYYKYDVGGFDYWGQGTLVTVSS

SEQ ID NO: 66 - protein, 121 aa, Artificial Sequence
  source: /note="Description of Artificial Sequence: Synthetic polypeptide"
QVQMVQSGAEVKKPGASVKVSCTASGFNIKDTYIHWVRQAPGQGLEWMGEIDPANDNTKYDPKFQGRVTITADTSTSTVYMELSSLRSEDTAVYYCATYYYKYDVGGFDYWGQGTLVTVSS

SEQ ID NO: 67 - protein, 121 aa, Artificial Sequence
  source: /note="Description of Artificial Sequence: Synthetic polypeptide"
QVQMKQSGAEVKKPGASVKVSCKASGFNIKDTYIHWVRQAPGQGLEWMGEIDPANDNTKYDPKFQGRVTITADTSTSTVYMELSSLRSEDTAVYYCATYYYKYDVGGFDYWGQGTLVTVSS

SEQ ID NO: 68 - protein, 121 aa, Artificial Sequence
  source: /note="Description of Artificial Sequence: Synthetic polypeptide"
QVQMKQSGAEVKKPGASVKVSCTASGFNIKDTYIHWVRQAPGQGLEWMGEIDPANDNTKYDPKFQGRVTITADTSTSTVYMELSSLRSEDTAVYYCATYYYKYDVGGFDYWGQGTLVTVSS

SEQ ID NO: 69 - protein, 121 aa, Artificial Sequence
  source: /note="Description of Artificial Sequence: Synthetic polypeptide"
QVQLKQSGAEVKKPGASVKVSCKASGFNIKDTYIHWVRQAPGQGLEWMGEIDPANDNTKYDPKFQGRVTITADTSTSTVYMELSSLRSEDTAVYYCATYYYKYDVGGFDYWGQGTLVTVSS

SEQ ID NO: 70 - protein, 121 aa, Artificial Sequence
  source: /note="Description of Artificial Sequence: Synthetic polypeptide"
QVQLKQSGAEVKKPGASVKVSCTASGFNIKDTYIHWVRQAPGQGLEWMGEIDPANDNTKYDPKFQGRVTITADTSTSTVYMELSSLRSEDTAVYYCATYYYKYDVGGFDYWGQGTLVTVSS

SEQ ID NO: 71 - protein, 121 aa, Artificial Sequence
  source: /note="Description of Artificial Sequence: Synthetic polypeptide"
QVQLVQSGAEVKKPGASVKVSCKASGFNIKDTYIHWVRQAPGQGLEWMGEIDPANDNTKYDPKFQGRVTITADTSSNTVYMELSSLRSEDTAVYYCATYYYKYDVGGFDYWGQGTLVTVSS

SEQ ID NO: 72 - protein, 121 aa, Artificial Sequence
  source: /note="Description of Artificial Sequence: Synthetic polypeptide"
QVQMKQSGAEVKKPGASVKVSCTASGFNIKDTYIHWVRQAPGQGLEWMGEIDPANDNTKYDPKFQGRVTITADTSSNTVYMELSSLRSEDTAVYYCATYYYKYDVGGFDYWGQGTLVTVSS

SEQ ID NO: 73 - protein, 108 aa, Artificial Sequence
  source: /note="Description of Artificial Sequence: Synthetic polypeptide"
EIVLTQSPGTLSLSPGERATLSCSVSSSISSSNLHWYQQKPGQAPRLLIYGTSNLASGIPDRFSGSGSGTDFTLTISRLEPEDFAVYYCQQWSSYPFTFGQGTKVEIK

SEQ ID NO: 74 - protein, 108 aa, Artificial Sequence
  source: /note="Description of Artificial Sequence: Synthetic polypeptide"
EIVLTQSPGTLSLSPGERATLSCSVSSSISSSNLHWYQQKPGQAPRLLIYGTSNLASGIPDRFSGSGSGTSYTLTISRLEPEDFAVYYCQQWSSYPFTFGQGTKVEIK

SEQ ID NO: 75 - protein, 108 aa, Artificial Sequence
  source: /note="Description of Artificial Sequence: Synthetic polypeptide"
EILLTQSPGTLSLSPGERATLSCSVSSSISSSNLHWFQQKPGQAPRLLIYGTSNLASGIPDRFSGSGSGTSYTLTISRLEPEDFAVYYCQQWSSYPFTFGQGTKVEIK

SEQ ID NO: 76 - protein, 108 aa, Artificial Sequence
  source: /note="Description of Artificial Sequence: Synthetic polypeptide"
EILLTQSPGTLSLSPGERATLSCSVSSSISSSNLHWFQQKPGQAPRLWIYGTSNLASGVPDRFSGSGSGTSYTLTISRLEPEDFAVYYCQQWSSYPFTFGQGTKVEIK

SEQ ID NO: 77 - protein, 108 aa, Artificial Sequence
  source: /note="Description of Artificial Sequence: Synthetic polypeptide"
EILLTQSPGTLSLSPGERATLTCSVSSSISSSNLHWFQQKPGQSPRLWIYGTSNLASGVPDRFSGSGSGTSYTLTISRLEPEDFAVYYCQQWSSYPFTFGQGTKVEIK

SEQ ID NO: 78 - protein, 5 aa, Artificial Sequence
  source: /note="Description of Artificial Sequence: Synthetic peptide"
DTYMY

SEQ ID NO: 79 - protein, 5 aa, Artificial Sequence
  source: /note="Description of Artificial Sequence: Synthetic peptide"
DTYIH

SEQ ID NO: 80 - protein, 5 aa, Artificial Sequence
  source: /note="Description of Artificial Sequence: Synthetic peptide"
DTYIY

SEQ ID NO: 81 - protein, 5 aa, Artificial Sequence
  source: /note="Description of Artificial Sequence: Synthetic peptide"
DNYIH

SEQ ID NO: 82 - protein, 5 aa, Artificial Sequence
  source: /note="Description of Artificial Sequence: Synthetic peptide"
DNYMD

SEQ ID NO: 83 - protein, 17 aa, Artificial Sequence
  source: /note="Description of Artificial Sequence: Synthetic peptide"
RIDPANGNTKYDPKLQG

SEQ ID NO: 84 - protein, 17 aa, Artificial Sequence
  source: /note="Description of Artificial Sequence: Synthetic peptide"
EIDPANGNTKYDPKFQG

SEQ ID NO: 85 - protein, 17 aa, Artificial Sequence
  source: /note="Description of Artificial Sequence: Synthetic peptide"
RIDPANGNTKFDPKFQG

SEQ ID NO: 86 - protein, 17 aa, Artificial Sequence
  source: /note="Description of Artificial Sequence: Synthetic peptide"
RIDPANGNTKFDPKFQD

SEQ ID NO: 87 - protein, 17 aa, Artificial Sequence
  source: /note="Description of Artificial Sequence: Synthetic peptide"
SIDPANGNTKYDPKFQG

SEQ ID NO: 88 - protein, 17 aa, Artificial Sequence
  source: /note="Description of Artificial Sequence: Synthetic peptide"
EIDPANGNSKYAPRFQG

SEQ ID NO: 89 - protein, 17 aa, Artificial Sequence
  source: /note="Description of Artificial Sequence: Synthetic peptide"
EIDPANGHTKYDPKFQG

SEQ ID NO: 90 - protein, 17 aa, Artificial Sequence
  source: /note="Description of Artificial Sequence: Synthetic peptide"
EIDPANDNTKYDPKFQG

SEQ ID NO: 91 - protein, 17 aa, Artificial Sequence
  source: /note="Description of Artificial Sequence: Synthetic peptide"
RIDPANGNTKYDPKFQG

SEQ ID NO: 92 - protein, 17 aa, Artificial Sequence
  source: /note="Description of Artificial Sequence: Synthetic peptide"
RIDPANGNTHFDPKFQG

SEQ ID NO: 93 - protein, 17 aa, Artificial Sequence
  source: /note="Description of Artificial Sequence: Synthetic peptide"
KIDPANGNTKYDPKFQG

SEQ ID NO: 94 - protein, 12 aa, Artificial Sequence
  source: /note="Description of Artificial Sequence: Synthetic peptide"
YSYRYDVGGFDY

SEQ ID NO: 95 - protein, 12 aa, Artificial Sequence
  source: /note="Description of Artificial Sequence: Synthetic peptide"
YYYRYDVGGFDY

SEQ ID NO: 96 - protein, 12 aa, Artificial Sequence
  source: /note="Description of Artificial Sequence: Synthetic peptide"
YFYRYDVGGFDY

SEQ ID NO: 97 - protein, 12 aa, Artificial Sequence
  source: /note="Description of Artificial Sequence: Synthetic peptide"
YFDKYDVGGCDY

SEQ ID NO: 98 - protein, 12 aa, Artificial Sequence
  source: /note="Description of Artificial Sequence: Synthetic peptide"
YYYKYDVGGFDY

SEQ ID NO: 99 - protein, 12 aa, Artificial Sequence
  source: /note="Description of Artificial Sequence: Synthetic peptide"
YYYRYEVGGFDY

SEQ ID NO: 100 - protein, 12 aa, Artificial Sequence
  source: /note="Description of Artificial Sequence: Synthetic peptide"
SVSSSISSSNLH

SEQ ID NO: 101 - protein, 12 aa, Artificial Sequence
  source: /note="Description of Artificial Sequence: Synthetic peptide"
SVSSSISSSTLH

SEQ ID NO: 102 - protein, 12 aa, Artificial Sequence
  source: /note="Description of Artificial Sequence: Synthetic peptide"
SVSSSISSSNLY

SEQ ID NO: 103 - protein, 12 aa, Artificial Sequence
  source: /note="Description of Artificial Sequence: Synthetic peptide"
SVSSGISSSNLH

SEQ ID NO: 104 - protein, 7 aa, Artificial Sequence
  source: /note="Description of Artificial Sequence: Synthetic peptide"
GTSNLAS

SEQ ID NO: 105 - protein, 9 aa, Artificial Sequence
  source: /note="Description of Artificial Sequence: Synthetic peptide"
QQWSSYPFT

SEQ ID NO: 106 - protein, 9 aa, Artificial Sequence
  source: /note="Description of Artificial Sequence: Synthetic peptide"
QQWNSYPLT

SEQ ID NO: 107 - protein, 9 aa, Artificial Sequence
  source: /note="Description of Artificial Sequence: Synthetic peptide"
QQWSSYPHT

SEQ ID NO: 108 - protein, 9 aa, Artificial Sequence
  source: /note="Description of Artificial Sequence: Synthetic peptide"
QQWSSYPWT

SEQ ID NO: 109 - protein, 9 aa, Artificial Sequence
  source: /note="Description of Artificial Sequence: Synthetic peptide"
QQWSSYPLT

SEQ ID NO: 110 - protein, 9 aa, Artificial Sequence
  source: /note="Description of Artificial Sequence: Synthetic peptide"
QQWSTYPFT

SEQ ID NO: 111 - protein, 9 aa, Artificial Sequence
  source: /note="Description of Artificial Sequence: Synthetic peptide"
QQWSRYPWT

SEQ ID NO: 112 - protein, 9 aa, Artificial Sequence
  source: /note="Description of Artificial Sequence: Synthetic peptide"
QQWRSYPFT

SEQ ID NO: 113 - protein, 30 aa, Artificial Sequence
  source: /note="Description of Artificial Sequence: Synthetic polypeptide"
QVQLVQSGAEVKKPGASVKVSCKASGFNIK

SEQ ID NO: 114 - protein, 30 aa, Artificial Sequence
  source: /note="Description of Artificial Sequence: Synthetic polypeptide"
QVQMKQSGAEVKKPGASVKVSCTASGFNIK

SEQ ID NO: 115 - protein, 30 aa, Artificial Sequence
  source: /note="Description of Artificial Sequence: Synthetic polypeptide"
QVQMKQSGAEVVKPGASVKVSCTASGFNIK

SEQ ID NO: 116 - protein, 30 aa, Artificial Sequence
  source: /note="Description of Artificial Sequence: Synthetic polypeptide"
QVQLVQSGAEVKKPGASVKVSCTASGFNIK

SEQ ID NO: 117 - protein, 30 aa, Artificial Sequence
  source: /note="Description of Artificial Sequence: Synthetic polypeptide"
QVQMVQSGAEVKKPGASVKVSCKASGFNIK

SEQ ID NO: 118 - protein, 30 aa, Artificial Sequence
  source: /note="Description of Artificial Sequence: Synthetic polypeptide"
QVQMVQSGAEVKKPGASVKVSCTASGFNIK

SEQ ID NO: 119 - protein, 30 aa, Artificial Sequence
  source: /note="Description of Artificial Sequence: Synthetic polypeptide"
QVQMKQSGAEVKKPGASVKVSCKASGFNIK

SEQ ID NO: 120 - protein, 30 aa, Artificial Sequence
  source: /note="Description of Artificial Sequence: Synthetic polypeptide"
QVQLKQSGAEVKKPGASVKVSCKASGFNIK

SEQ ID NO: 121 - protein, 30 aa, Artificial Sequence
  source: /note="Description of Artificial Sequence: Synthetic polypeptide"
QVQLKQSGAEVKKPGASVKVSCTASGFNIK

SEQ ID NO: 122 - protein, 14 aa, Artificial Sequence
  source: /note="Description of Artificial Sequence: Synthetic peptide"
WVRQAPGQGLEWMG

SEQ ID NO: 123 - protein, 14 aa, Artificial Sequence
  source: /note="Description of Artificial Sequence: Synthetic peptide"
WVRQAPGQGLEWIG

SEQ ID NO: 124 - protein, 32 aa, Artificial Sequence
  source: /note="Description of Artificial Sequence: Synthetic polypeptide"
RVTMTRDTSTSTVYMELSSLRSEDTAVYYCAR

SEQ ID NO: 125 - protein, 32 aa, Artificial Sequence
  source: /note="Description of Artificial Sequence: Synthetic polypeptide"
RVTITADTSTSTVYMELSSLRSEDTAVYYCAT

SEQ ID NO: 126 - protein, 32 aa, Artificial Sequence
  source: /note="Description of Artificial Sequence: Synthetic polypeptide"
RVTITADTSSNTVYMELSSLRSEDTAVYYCAT

SEQ ID NO: 127 - protein, 32 aa, Artificial Sequence
  source: /note="Description of Artificial Sequence: Synthetic polypeptide"
RVTITADTSSNTVYLQLSSLRSEDTAVYYCAT

SEQ ID NO: 128 - protein, 11 aa, Artificial Sequence
  source: /note="Description of Artificial Sequence: Synthetic peptide"
WGQGTLVTVSS

SEQ ID NO: 129 - protein, 23 aa, Artificial Sequence
  source: /note="Description of Artificial Sequence: Synthetic peptide"
EIVLTQSPGTLSLSPGERATLSC

SEQ ID NO: 130 - protein, 23 aa, Artificial Sequence
  source: /note="Description of Artificial Sequence: Synthetic peptide"
EILLTQSPGTLSLSPGERATLSC

SEQ ID NO: 131 - protein, 23 aa, Artificial Sequence
  source: /note="Description of Artificial Sequence: Synthetic peptide"
EILLTQSPGTLSLSPGERATLTC

SEQ ID NO: 132 - protein, 15 aa, Artificial Sequence
  source: /note="Description of Artificial Sequence: Synthetic peptide"
WYQQKPGQAPRLLIY

SEQ ID NO: 133 - protein, 15 aa, Artificial Sequence
  source: /note="Description of Artificial Sequence: Synthetic peptide"
WFQQKPGQAPRLLIY

SEQ ID NO: 134 - protein, 15 aa, Artificial Sequence
  source: /note="Description of Artificial Sequence: Synthetic peptide"
WFQQKPGQAPRLWIY

SEQ ID NO: 135 - protein, 15 aa, Artificial Sequence
  source: /note="Description of Artificial Sequence: Synthetic peptide"
WFQQKPGQSPRLWIY

SEQ ID NO: 136 - protein, 32 aa, Artificial Sequence
  source: /note="Description of Artificial Sequence: Synthetic polypeptide"
GIPDRFSGSGSGTDFTLTISRLEPEDFAVYYC

SEQ ID NO: 137 - protein, 32 aa, Artificial Sequence
  source: /note="Description of Artificial Sequence: Synthetic polypeptide"
GIPDRFSGSGSGTSYTLTISRLEPEDFAVYYC

SEQ ID NO: 138 - protein, 32 aa, Artificial Sequence
  source: /note="Description of Artificial Sequence: Synthetic polypeptide"
GVPDRFSGSGSGTSYTLTISRLEPEDFAVYYC

SEQ ID NO: 139 - protein, 10 aa, Artificial Sequence
  source: /note="Description of Artificial Sequence: Synthetic peptide"
FGQGTKVEIK

SEQ ID NO: 140 - protein, 5 aa, Artificial Sequence
  source: /note="Description of Artificial Sequence: Synthetic peptide"
  VARIANT (2)..(2): /replace="N"
  VARIANT (4)..(4): /replace="M"
  VARIANT (5)..(5): /replace="Y" or "D"
  MISC_FEATURE (1)..(5): /note="Variant residues given in the sequence have no preference with respect to those in the annotations for variant positions"
DTYIH

SEQ ID NO: 141 - protein, 5 aa, Artificial Sequence
  source: /note="Description of Artificial Sequence: Synthetic peptide"
  VARIANT (2)..(2): /replace="N"
  VARIANT (4)..(4): /replace="M"
  VARIANT (5)..(5): /replace="Y"
  MISC_FEATURE (1)..(5): /note="Variant residues given in the sequence have no preference with respect to those in the annotations for variant positions"
DTYIH

SEQ ID NO: 142 - protein, 17 aa, Artificial Sequence
  source: /note="Description of Artificial Sequence: Synthetic peptide"
  VARIANT (1)..(1): /replace="R" or "S" or "K"
  VARIANT (7)..(7): /replace="G"
  VARIANT (8)..(8): /replace="H"
  VARIANT (9)..(9): /replace="S"
  VARIANT (10)..(10): /replace="H"
  VARIANT (11)..(11): /replace="F"
  VARIANT (12)..(12): /replace="A"
  VARIANT (14)..(14): /replace="R"
  VARIANT (15)..(15): /replace="L"
  VARIANT (17)..(17): /replace="D"
  MISC_FEATURE (1)..(17): /note="Variant residues given in the sequence have no preference with respect to those in the annotations for variant positions"
EIDPANDNTKYDPKFQG

SEQ ID NO: 143 - protein, 17 aa, Artificial Sequence
  source: /note="Description of Artificial Sequence: Synthetic peptide"
  VARIANT (1)..(1): /replace="R" or "S"
  VARIANT (7)..(7): /replace="G"
  VARIANT (8)..(8): /replace="H"
  VARIANT (9)..(9): /replace="S"
  VARIANT (11)..(11): /replace="F"
  VARIANT (12)..(12): /replace="A"
  VARIANT (14)..(14): /replace="R"
  VARIANT (17)..(17): /replace="D"
  MISC_FEATURE (1)..(17): /note="Variant residues given in the sequence have no preference with respect to those in the annotations for variant positions"
EIDPANDNTKYDPKFQG

SEQ ID NO: 144 - protein, 12 aa, Artificial Sequence
  source: /note="Description of Artificial Sequence: Synthetic peptide"
  VARIANT (2)..(2): /replace="F" or "S"
  VARIANT (3)..(3): /replace="D"
  VARIANT (4)..(4): /replace="R"
  VARIANT (6)..(6): /replace="E"
  VARIANT (10)..(10): /replace="C"
  MISC_FEATURE (1)..(12): /note="Variant residues given in the sequence have no preference with respect to those in the annotations for variant positions"
YYYKYDVGGFDY

SEQ ID NO: 145 - protein, 12 aa, Artificial Sequence
  source: /note="Description of Artificial Sequence: Synthetic peptide"
  VARIANT (2)..(2): /replace="F" or "S"
  VARIANT (3)..(3): /replace="D"
  VARIANT (4)..(4): /replace="R"
  VARIANT (10)..(10): /replace="C"
  MISC_FEATURE (1)..(12): /note="Variant residues given in the sequence have no preference with respect to those in the annotations for variant positions"
YYYKYDVGGFDY

SEQ ID NO: 146 - protein, 12 aa, Artificial Sequence
  source: /note="Description of Artificial Sequence: Synthetic peptide"
  VARIANT (4)..(4): /replace="R"
  VARIANT (6)..(6): /replace="E"
  MISC_FEATURE (1)..(12): /note="Variant residues given in the sequence have no preference with respect to those in the annotations for variant positions"
YYYKYDVGGFDY

SEQ ID NO: 147 - protein, 12 aa, Artificial Sequence
  source: /note="Description of Artificial Sequence: Synthetic peptide"
  VARIANT (5)..(5): /replace="G"
  VARIANT (10)..(10): /replace="T"
  VARIANT (12)..(12): /replace="Y"
  MISC_FEATURE (1)..(12): /note="Variant residues given in the sequence have no preference with respect to those in the annotations for variant positions"
SVSSSISSSNLH

SEQ ID NO: 148 - protein, 12 aa, Artificial Sequence
  source: /note="Description of Artificial Sequence: Synthetic peptide"
  VARIANT (12)..(12): /replace="Y"
  MISC_FEATURE (1)..(12): /note="Variant residues given in the sequence have no preference with respect to those in the annotations for variant positions"
SVSSSISSSNLH

SEQ ID NO: 149 - protein, 9 aa, Artificial Sequence
  source: /note="Description of Artificial Sequence: Synthetic peptide"
  VARIANT (4)..(4): /replace="N" or "R"
  VARIANT (5)..(5): /replace="T" or "R"
  VARIANT (8)..(8): /replace="L" or "H" or "W"
  MISC_FEATURE (1)..(9): /note="Variant residues given in the sequence have no preference with respect to those in the annotations for variant positions"
QQWSSYPFT

SEQ ID NO: 150 - protein, 9 aa, Artificial Sequence
  source: /note="Description of Artificial Sequence: Synthetic peptide"
  VARIANT (4)..(4): /replace="N" or "R"
  VARIANT (8)..(8): /replace="L" or "H"
  MISC_FEATURE (1)..(9): /note="Variant residues given in the sequence have no preference with respect to those in the annotations for variant positions"
QQWSSYPFT

SEQ ID NO: 151 - protein, 121 aa, Artificial Sequence; identical to SEQ ID NO: 65
  source: /note="Description of Artificial Sequence: Synthetic polypeptide"
  VARIANT (4)..(4): /replace="L"
  VARIANT (5)..(5): /replace="K"
  VARIANT (12)..(12): /replace="V"
  VARIANT (48)..(48): /replace="I"
  VARIANT (70)..(70): /replace="M"
  VARIANT (72)..(72): /replace="R"
  VARIANT (76)..(76): /replace="S"
  VARIANT (77)..(77): /replace="N"
  VARIANT (81)..(81): /replace="L"
  VARIANT (82)..(82): /replace="Q"
  VARIANT (98)..(98): /replace="R"
  VARIANT (102)..(102): /replace="R"
  VARIANT (104)..(104): /replace="E"
  MISC_FEATURE (1)..(121): /note="Variant residues given in the sequence have no preference with respect to those in the annotations for variant positions"

SEQ ID NO: 152 - protein, 108 aa, Artificial Sequence; identical to SEQ ID NO: 73
  source: /note="Description of Artificial Sequence: Synthetic polypeptide"
  VARIANT (3)..(3): /replace="L"
  VARIANT (22)..(22): /replace="T"
  VARIANT (37)..(37): /replace="F"
  VARIANT (44)..(44): /replace="S"
  VARIANT (48)..(48): /replace="W"
  VARIANT (59)..(59): /replace="V"
  VARIANT (71)..(71): /replace="S"
  VARIANT (72)..(72): /replace="Y"
  MISC_FEATURE (1)..(108): /note="Variant residues given in the sequence have no preference with respect to those in the annotations for variant positions"

SEQ ID NO: 153 - protein, 98 aa, Homo sapiens
QVQLVQSGAEVKKPGASVKVSCKASGYTFTSYYMHWVRQAPGQGLEWMGIINPSGGSTSYAQKFQGRVTMTRDTSTSTVYMELSSLRSEDTAVYYCAR

SEQ ID NO: 154 - protein, 98 aa, Homo sapiens
EVQLVQSGAEVKKPGATVKISCKVSGYTFTDYYMHWVQQAPGKGLEWMGLVDPEDGETIYAEKFQGRVTITADTSTDTAYMELSSLRSEDTAVYYCAT

SEQ ID NO: 155 - protein, 98 aa, Homo sapiens
QVQLVQSGAEVKKPGASVKVSCKASGYTFTSYAMHWVRQAPGQRLEWMGWINAGNGNTKYSQKFQGRVTITRDTSASTAYMELSSLRSEDTAVYYCAR

SEQ ID NO: 156 - protein, 98 aa, Homo sapiens
QVQLVQSGAEVKKPGASVKVSCKVSGYTLTELSMHWVRQAPGKGLEWMGGFDPEDGETIYAQKFQGRVTMTEDTSTDTAYMELSSLRSEDTAVYYCAT

SEQ ID NO: 157 - protein, 98 aa, Homo sapiens
QVQLVQSGAEVKKPGASVKVSCKASGYTFTGYYMHWVRQAPGQGLEWMGRINPNSGGTNYAQKFQGRVTSTRDTSISTAYMELSRLRSDDTVVYYCAR

SEQ ID NO: 158 - protein, 98 aa, Homo sapiens
QMQLVQSGAEVKKTGSSVKVSCKASGYTFTYRYLHWVRQAPGQALEWMGWITPFNGNTNYAQKFQDRVTITRDRSMSTAYMELSSLRSEDTAMYYCAR

SEQ ID NO: 159 - protein, 98 aa, Homo sapiens
QVQLVQSGAEVKKPGASVKVSCKASGYTFTSYGISWVRQAPGQGLEWMGWISAYNGNTNYAQKLQGRVTMTTDTSTSTAYMELRSLRSDDTAVYYCAR

SEQ ID NO: 160 - protein, 96 aa, Homo sapiens
EIVLTQSPGTLSLSPGERATLSCRASQSVSSSYLAWYQQKPGQAPRLLIYGASSRATGIPDRFSGSGSGTDFTLTISRLEPEDFAVYYCQQYGSSP

SEQ ID NO: 161 - protein, 95 aa, Homo sapiens
EIVMTQSPATLSVSPGERATLSCRASQSVSSNLAWYQQKPGQAPRLLIYGASTRATGIPARFSGSGSGTEFTLTISSLQSEDFAVYYCQQYNNWP

SEQ ID NO: 162 - protein, 96 aa, Homo sapiens
EIVLTQSPATLSLSPGERATLSCGASQSVSSSYLAWYQQKPGLAPRLLIYDASSRATGIPDRFSGSGSGTDFTLTISRLEPEDFAVYYCQQYGSSP

SEQ ID NO: 163 - protein, 97 aa, Homo sapiens
EIVMTQSPATLSLSPGERATLSCRASQSVSSSYLSWYQQKPGQAPRLLIYGASTRATGIPARFSGSGSGTDFTLTISSLQPEDFAVYYCQQDYNLPP

SEQ ID NO: 164 - protein, 95 aa, Homo sapiens
DIQLTQSPSFLSASVGDRVTITCRASQGISSYLAWYQQKPGKAPKLLIYAASTLQSGVPSRFSGSGSGTEFTLTISSLQPEDFATYYCQQLNSYP

SEQ ID NO: 165 - protein, 95 aa, Homo sapiens
EIVLTQSPATLSLSPGERATLSCRASQSVSSYLAWYQQKPGQAPRLLIYDASNRATGIPARFSGSGSGTDFTLTISSLEPEDFAVYYCQQRSNWP

SEQ ID NO: 166 - protein, 525 aa, Homo sapiens
MWEAQFLGLLFLQPLWVAPVKPLQPGAEVPVVWAQEGAPAQLPCSPTIPLQDLSLLRRAGVTWQHQPDSGPPAAAPGHPLAPGPHPAAPSSWGPRPRRYTVLSVGPGGLRSGRLPLQPRVQLDERGRQRGDFSLWLRPARRADAGEYRAAVHLRDRALSCRLRLRLGQASMTASPPGSLRASDWVILNCSFSRPDRPASVHWFRNRGQGRVPVRESPHHHLAESFLFLPQVSPMDSGPWGCILTYRDGFNVSIMYNLTVLGLEPPTPLTVYAGAGSRVGLPCRLPAGVGTRSFLTAKWTPPGGGPDLLVTGDNGDFTLRLEDVSQAQAGTYTCHIHLQEQQLNATVTLAIITVTPKSFGSPGSLGKLLCEVTPVSGQERFVWSSLDTPSQRSFSGPWLEAQEAQLLSQPWQCQLYQGERLLGAAVYFTELSSPGAQRSGRAPGALPAGHLLLFLILGVLSLLLLVTGAFGFHLWRRQWRPRRFSALEQGIHPPQAQSKIEELEQEPEPEPEPEPEPEPEPEPEQL

SEQ ID NO: 167 - protein, 497 aa, Homo sapiens
VPVVWAQEGAPAQLPCSPTIPLQDLSLLRRAGVTWQHQPDSGPPAAAPGHPLAPGPHPAAPSSWGPRPRRYTVLSVGPGGLRSGRLPLQPRVQLDERGRQRGDFSLWLRPARRADAGEYRAAVHLRDRALSCRLRLRLGQASMTASPPGSLRASDWVILNCSFSRPDRPASVHWFRNRGQGRVPVRESPHHHLAESFLFLPQVSPMDSGPWGCILTYRDGFNVSIMYNLTVLGLEPPTPLTVYAGAGSRVGLPCRLPAGVGTRSFLTAKWTPPGGGPDLLVTGDNGDFTLRLEDVSQAQAGTYTCHIHLQEQQLNATVTLAIITVTPKSFGSPGSLGKLLCEVTPVSGQERFVWSSLDTPSQRSFSGPWLEAQEAQLLSQPWQCQLYQGERLLGAAVYFTELSSPGAQRSGRAPGALPAGHLLLFLILGVLSLLLLVTGAFGFHLWRRQWRPRRFSALEQGIHPPQAQSKIEELEQEPEPEPEPEPEPEPEPEPEQL

SEQ ID NO: 168 - protein, 450 aa, Artificial Sequence
  source: /note="Description of Artificial Sequence: Synthetic polypeptide"
QVQMVQSGAEVKKPGASVKVSCKASGFNIKDTYIHWVRQAPGQGLEWMGEIDPANDNTKYDPKFQGRVTITADTSTSTVYMELSSLRSEDTAVYYCATYYYKYDVGGFDYWGQGTLVTVSSASTKGPSVFPLAPSSKSTSGGTAALGCLVKDYFPEPVTVSWNSGALTSGVHTFPAVLQSSGLYSLSSVVTVPSSSLGTQTYICNVNHKPSNTKVDKRVEPKSCDKTHTCPPCPAPELLGGPSVFLFPPKPKDTLMISRTPEVTCVVVDVSHEDPEVKFNWYVDGVEVHNAKTKPREEQYNSTYRVVSVLTVLHQDWLNGKEYKCKVSNKALPAPIEKTISKAKGQPREPQVYTLPPSREEMTKNQVSLTCLVKGFYPSDIAVEWESNGQPENNYKTTPPVLDSDGSFFLYSKLTVDKSRWQQGNVFSCSVMHEALHNHYTQKSLSLSPG

SEQ ID NO: 169 - protein, 450 aa, Artificial Sequence
  source: /note="Description of Artificial Sequence: Synthetic polypeptide"
QVQMVQSGAEVKKPGASVKVSCKASGFNIKDTYIHWVRQAPGQGLEWMGEIDPANDNTKYDPKFQGRVTITADTSTSTVYMELSSLRSEDTAVYYCATYYYKYDVGGFDYWGQGTLVTVSSASTKGPSVFPLAPSSKSTSGGTAALGCLVKDYFPEPVTVSWNSGALTSGVHTFPAVLQSSGLYSLSSVVTVPSSSLGTQTYICNVNHKPSNTKVDKRVEPKSCDKTHTCPPCPAPELLGGPSVFLFPPKPKDTLMISRTPEVTCVVVDVSHEDPEVKFNWYVDGVEVHNAKTKPREEQYASTYRVVSVLTVLHQDWLNGKEYKCKVSNKALPAPIEKTISKAKGQPREPQVYTLPPSREEMTKNQVSLTCLVKGFYPSDIAVEWESNGQPENNYKTTPPVLDSDGSFFLYSKLTVDKSRWQQGNVFSCSVMHEALHNHYTQKSLSLSPG

SEQ ID NO: 170 - protein, 447 aa, Artificial Sequence
  source: /note="Description of Artificial Sequence: Synthetic polypeptide"
QVQMVQSGAEVKKPGASVKVSCKASGFNIKDTYIHWVRQAPGQGLEWMGEIDPANDNTKYDPKFQGRVTITADTSTSTVYMELSSLRSEDTAVYYCATYYYKYDVGGFDYWGQGTLVTVSSASTKGPSVFPLAPCSRSTSESTAALGCLVKDYFPEPVTVSWNSGALTSGVHTFPAVLQSSGLYSLSSVVTVPSSSLGTKTYTCNVDHKPSNTKVDKRVESKYGPPCPPCPAPEFLGGPSVFLFPPKPKDTLMISRTPEVTCVVVDVSQEDPEVQFNWYVDGVEVHNAKTKPREEQFNSTYRVVSVLTVLHQDWLNGKEYKCKVSNKGLPSSIEKTISKAKGQPREPQVYTLPPSQEEMTKNQVSLTCLVKGFYPSDIAVEWESNGQPENNYKTTPPVLDSDGSFFLYSRLTVDKSRWQEGNVFSCSVMHEALHNHYTQKSLSLSLG

SEQ ID NO: 171 - protein, 450 aa, Artificial Sequence
  source: /note="Description of Artificial Sequence: Synthetic polypeptide"
QVQLVQSGAEVKKPGASVKVSCKASGFNIKDTYIHWVRQAPGQGLEWMGEIDPANDNTKYDPKFQGRVTMTRDTSTSTVYMELSSLRSEDTAVYYCARYYYRYDVGGFDYWGQGTLVTVSSASTKGPSVFPLAPSSKSTSGGTAALGCLVKDYFPEPVTVSWNSGALTSGVHTFPAVLQSSGLYSLSSVVTVPSSSLGTQTYICNVNHKPSNTKVDKRVEPKSCDKTHTCPPCPAPELLGGPSVFLFPPKPKDTLMISRTPEVTCVVVDVSHEDPEVKFNWYVDGVEVHNAKTKPREEQYASTYRVVSVLTVLHQDWLNGKEYKCKVSNKALPAPIEKTISKAKGQPREPQVYTLPPSREEMTKNQVSLTCLVKGFYPSDIAVEWESNGQPENNYKTTPPVLDSDGSFFLYSKLTVDKSRWQQGNVFSCSVMHEALHNHYTQKSLSLSPG

SEQ ID NO: 172 - protein, 450 aa, Artificial Sequence
  source: /note="Description of Artificial Sequence: Synthetic polypeptide"
QVQLVQSGAEVKKPGASVKVSCKASGFNIKDTYIHWVRQAPGQGLEWMGEIDPANDNTKYDPKFQGRVTITADTSTSTVYMELSSLRSEDTAVYYCATYYYRYDVGGFDYWGQGTLVTVSSASTKGPSVFPLAPSSKSTSGGTAALGCLVKDYFPEPVTVSWNSGALTSGVHTFPAVLQSSGLYSLSSVVTVPSSSLGTQTYICNVNHKPSNTKVDKRVEPKSCDKTHTCPPCPAPELLGGPSVFLFPPKPKDTLMISRTPEVTCVVVDVSHEDPEVKFNWYVDGVEVHNAKTKPREEQYASTYRVVSVLTVLHQDWLNGKEYKCKVSNKALPAPIEKTISKAKGQPREPQVYTLPPSREEMTKNQVSLTCLVKGFYPSDIAVEWESNGQPENNYKTTPPVLDSDGSFFLYSKLTVDKSRWQQGNVFSCSVMHEALHNHYTQKSLSLSPG

SEQ ID NO: 173 - protein, 450 aa, Artificial Sequence
  source: /note="Description of Artificial Sequence: Synthetic polypeptide"
QVQLVQSGAEVKKPGASVKVSCKASGFNIKDTYIHWVRQAPGQGLEWMGEIDPANDNTKYDPKFQGRVTITADTSSNTVYMELSSLRSEDTAVYYCATYYYRYDVGGFDYWGQGTLVTVSSASTKGPSVFPLAPSSKSTSGGTAALGCLVKDYFPEPVTVSWNSGALTSGVHTFPAVLQSSGLYSLSSVVTVPSSSLGTQTYICNVNHKPSNTKVDKRVEPKSCDKTHTCPPCPAPELLGGPSVFLFPPKPKDTLMISRTPEVTCVVVDVSHEDPEVKFNWYVDGVEVHNAKTKPREEQYASTYRVVSVLTVLHQDWLNGKEYKCKVSNKALPAPIEKTISKAKGQPREPQVYTLPPSREEMTKNQVSLTCLVKGFYPSDIAVEWESNGQPENNYKTTPPVLDSDGSFFLYSKLTVDKSRWQQGNVFSCSVMHEALHNHYTQKSLSLSPG

SEQ ID NO: 174 - protein, 450 aa, Artificial Sequence
  source: /note="Description of Artificial Sequence: Synthetic polypeptide"
QVQMKQSGAEVKKPGASVKVSCTASGFNIKDTYIHWVRQAPGQGLEWMGEIDPANDNTKYDPKFQGRVTITADTSSNTVYMELSSLRSEDTAVYYCATYYYRYDVGGFDYWGQGTLVTVSSASTKGPSVFPLAPSSKSTSGGTAALGCLVKDYFPEPVTVSWNSGALTSGVHTFPAVLQSSGLYSLSSVVTVPSSSLGTQTYICNVNHKPSNTKVDKRVEPKSCDKTHTCPPCPAPELLGGPSVFLFPPKPKDTLMISRTPEVTCVVVDVSHEDPEVKFNWYVDGVEVHNAKTKPREEQYASTYRVVSVLTVLHQDWLNGKEYKCKVSNKALPAPIEKTISKAKGQPREPQVYTLPPSREEMTKNQVSLTCLVKGFYPSDIAVEWESNGQPENNYKTTPPVLDSDGSFFLYSKLTVDKSRWQQGNVFSCSVMHEALHNHYTQKSLSLSPG

SEQ ID NO: 175 - protein, 450 aa, Artificial Sequence
  source: /note="Description of Artificial Sequence: Synthetic polypeptide"
QVQMKQSGAEVVKPGASVKVSCTASGFNIKDTYIHWVRQAPGQGLEWIGEIDPANDNTKYDPKFQGRVTITADTSSNTVYLQLSSLRSEDTAVYYCATYYYRYDVGGFDYWGQGTLVTVSSASTKGPSVFPLAPSSKSTSGGTAALGCLVKDYFPEPVTVSWNSGALTSGVHTFPAVLQSSGLYSLSSVVTVPSSSLGTQTYICNVNHKPSNTKVDKRVEPKSCDKTHTCPPCPAPELLGGPSVFLFPPKPKDTLMISRTPEVTCVVVDVSHEDPEVKFNWYVDGVEVHNAKTKPREEQYASTYRVVSVLTVLHQDWLNGKEYKCKVSNKALPAPIEKTISKAKGQPREPQVYTLPPSREEMTKNQVSLTCLVKGFYPSDIAVEWESNGQPENNYKTTPPVLDSDGSFFLYSKLTVDKSRWQQGNVFSCSVMHEALHNHYTQKSLSLSPG

SEQ ID NO: 176 - protein, 450 aa, Artificial Sequence
  source: /note="Description of Artificial Sequence: Synthetic polypeptide"
QVQMKQSGAEVVKPGASVKVSCTASGFNIKDTYIHWVRQAPGQGLEWIGEIDPANDNTKYDPKFQGRVTITADTSSNTVYLQLSSLRSEDTAVYYCATYYYKYDVGGFDYWGQGTLVTVSSASTKGPSVFPLAPSSKSTSGGTAALGCLVKDYFPEPVTVSWNSGALTSGVHTFPAVLQSSGLYSLSSVVTVPSSSLGTQTYICNVNHKPSNTKVDKRVEPKSCDKTHTCPPCPAPELLGGPSVFLFPPKPKDTLMISRTPEVTCVVVDVSHEDPEVKFNWYVDGVEVHNAKTKPREEQYASTYRVVSVLTVLHQDWLNGKEYKCKVSNKALPAPIEKTISKAKGQPREPQVYTLPPSREEMTKNQVSLTCLVKGFYPSDIAVEWESNGQPENNYKTTPPVLDSDGSFFLYSKLTVDKSRWQQGNVFSCSVMHEALHNHYTQKSLSLSPG

SEQ ID NO: 177 - protein, 450 aa, Artificial Sequence
  source: /note="Description of Artificial Sequence: Synthetic polypeptide"
QVQMKQSGAEVVKPGASVKVSCTASGFNIKDTYIHWVRQAPGQGLEWIGEIDPANDNTKYDPKFQGRVTITADTSSNTVYLQLSSLRSEDTAVYYCATYYYRYEVGGFDYWGQGTLVTVSSASTKGPSVFPLAPSSKSTSGGTAALGCLVKDYFPEPVTVSWNSGALTSGVHTFPAVLQSSGLYSLSSVVTVPSSSLGTQTYICNVNHKPSNTKVDKRVEPKSCDKTHTCPPCPAPELLGGPSVFLFPPKPKDTLMISRTPEVTCVVVDVSHEDPEVKFNWYVDGVEVHNAKTKPREEQYASTYRVVSVLTVLHQDWLNGKEYKCKVSNKALPAPIEKTISKAKGQPREPQVYTLPPSREEMTKNQVSLTCLVKGFYPSDIAVEWESNGQPENNYKTTPPVLDSDGSFFLYSKLTVDKSRWQQGNVFSCSVMHEALHNHYTQKSLSLSPG

SEQ ID NO: 178 - protein, 450 aa, Artificial Sequence
  source: /note="Description of Artificial Sequence: Synthetic polypeptide"
QVQLVQSGAEVKKPGASVKVSCKASGFNIKDTYIHWVRQAPGQGLEWMGEIDPANDNTKYDPKFQGRVTITADTSTSTVYMELSSLRSEDTAVYYCATYYYKYDVGGFDYWGQGTLVTVSSASTKGPSVFPLAPSSKSTSGGTAALGCLVKDYFPEPVTVSWNSGALTSGVHTFPAVLQSSGLYSLSSVVTVPSSSLGTQTYICNVNHKPSNTKVDKRVEPKSCDKTHTCPPCPAPELLGGPSVFLFPPKPKDTLMISRTPEVTCVVVDVSHEDPEVKFNWYVDGVEVHNAKTKPREEQYASTYRVVSVLTVLHQDWLNGKEYKCKVSNKALPAPIEKTISKAKGQPREPQVYTLPPSREEMTKNQVSLTCLVKGFYPSDIAVEWESNGQPENNYKTTPPVLDSDGSFFLYSKLTVDKSRWQQGNVFSCSVMHEALHNHYTQKSLSLSPG

SEQ ID NO: 179 - protein, 450 aa, Artificial Sequence
  source: /note="Description of Artificial Sequence: Synthetic polypeptide"
QVQLVQSGAEVKKPGASVKVSCTASGFNIKDTYIHWVRQAPGQGLEWMGEIDPANDNTKYDPKFQGRVTITADTSTSTVYMELSSLRSEDTAVYYCATYYYKYDVGGFDYWGQGTLVTVSSASTKGPSVFPLAPSSKSTSGGTAALGCLVKDYFPEPVTVSWNSGALTSGVHTFPAVLQSSGLYSLSSVVTVPSSSLGTQTYICNVNHKPSNTKVDKRVEPKSCDKTHTCPPCPAPELLGGPSVFLFPPKPKDTLMISRTPEVTCVVVDVSHEDPEVKFNWYVDGVEVHNAKTKPREEQYASTYRVVSVLTVLHQDWLNGKEYKCKVSNKALPAPIEKTISKAKGQPREPQVYTLPPSREEMTKNQVSLTCLVKGFYPSDIAVEWESNGQPENNYKTTPPVLDSDGSFFLYSKLTVDKSRWQQGNVFSCSVMHEALHNHYTQKSLSLSPG

SEQ ID NO: 180 - protein, 450 aa, Artificial Sequence
  source: /note="Description of Artificial Sequence: Synthetic polypeptide"
QVQMVQSGAEVKKPGASVKVSCTASGFNIKDTYIHWVRQAPGQGLEWMGEIDPANDNTKYDPKFQGRVTITADTSTSTVYMELSSLRSEDTAVYYCATYYYKYDVGGFDYWGQGTLVTVSSASTKGPSVFPLAPSSKSTSGGTAALGCLVKDYFPEPVTVSWNSGALTSGVHTFPAVLQSSGLYSLSSVVTVPSSSLGTQTYICNVNHKPSNTKVDKRVEPKSCDKTHTCPPCPAPELLGGPSVFLFPPKPKDTLMISRTPEVTCVVVDVSHEDPEVKFNWYVDGVEVHNAKTKPREEQYASTYRVVSVLTVLHQDWLNGKEYKCKVSNKALPAPIEKTISKAKGQPREPQVYTLPPSREEMTKNQVSLTCLVKGFYPSDIAVEWESNGQPENNYKTTPPVLDSDGSFFLYSKLTVDKSRWQQGNVFSCSVMHEALHNHYTQKSLSLSPG

SEQ ID NO: 181 - protein, 450 aa, Artificial Sequence
  source: /note="Description of Artificial Sequence: Synthetic polypeptide"
QVQMKQSGAEVKKPGASVKVSCKASGFNIKDTYIHWVRQAPGQGLEWMGEIDPANDNTKYDPKFQGRVTITADTSTSTVYMELSSLRSEDTAVYYCATYYYKYDVGGFDYWGQGTLVTVSSASTKGPSVFPLAPSSKSTSGGTAALGCLVKDYFPEPVTVSWNSGALTSGVHTFPAVLQSSGLYSLSSVVTVPSSSLGTQTYICNVNHKPSNTKVDKRVEPKSCDKTHTCPPCPAPELLGGPSVFLFPPKPKDTLMISRTPEVTCVVVDVSHEDPEVKFNWYVDGVEVHNAKTKPREEQYASTYRVVSVLTVLHQDWLNGKEYKCKVSNKALPAPIEKTISKAKGQPREPQVYTLPPSREEMTKNQVSLTCLVKGFYPSDIAVEWESNGQPENNYKTTPPVLDSDGSFFLYSKLTVDKSRWQQGNVFSCSVMHEALHNHYTQKSLSLSPG

SEQ ID NO: 182 - protein, 450 aa, Artificial Sequence
  source: /note="Description of Artificial Sequence: Synthetic polypeptide"
QVQMKQSGAEVKKPGASVKVSCTASGFNIKDTYIHWVRQAPGQGLEWMGEIDPANDNTKYDPKFQGRVTITADTSTSTVYMELSSLRSEDTAVYYCATYYYKYDVGGFDYWGQGTLVTVSSASTKGPSVFPLAPSSKSTSGGTAALGCLVKDYFPEPVTVSWNSGALTSGVHTFPAVLQSSGLYSLSSVVTVPSSSLGTQTYICNVNHKPSNTKVDKRVEPKSCDKTHTCPPCPAPELLGGPSVFLFPPKPKDTLMISRTPEVTCVVVDVSHEDPEVKFNWYVDGVEVHNAKTKPREEQYASTYRVVSVLTVLHQDWLNGKEYKCKVSNKALPAPIEKTISKAKGQPREPQVYTLPPSREEMTKNQVSLTCLVKGFYPSDIAVEWESNGQPENNYKTTPPVLDSDGSFFLYSKLTVDKSRWQQGNVFSCSVMHEALHNHYTQKSLSLSPG

SEQ ID NO: 183 - protein, 450 aa, Artificial Sequence
  source: /note="Description of Artificial Sequence: Synthetic polypeptide"
QVQLKQSGAEVKKPGASVKVSCKASGFNIKDTYIHWVRQAPGQGLEWMGEIDPANDNTKYDPKFQGRVTITADTSTSTVYMELSSLRSEDTAVYYCATYYYKYDVGGFDYWGQGTLVTVSSASTKGPSVFPLAPSSKSTSGGTAALGCLVKDYFPEPVTVSWNSGALTSGVHTFPAVLQSSGLYSLSSVVTVPSSSLGTQTYICNVNHKPSNTKVDKRVEPKSCDKTHTCPPCPAPELLGGPSVFLFPPKPKDTLMISRTPEVTCVVVDVSHEDPEVKFNWYVDGVEVHNAKTKPREEQYASTYRVVSVLTVLHQDWLNGKEYKCKVSNKALPAPIEKTISKAKGQPREPQVYTLPPSREEMTKNQVSLTCLVKGFYPSDIAVEWESNGQPENNYKTTPPVLDSDGSFFLYSKLTVDKSRWQQGNVFSCSVMHEALHNHYTQKSLSLSPG

SEQ ID NO: 184 - protein, 450 aa, Artificial Sequence
  source: /note="Description of Artificial Sequence: Synthetic polypeptide"
QVQLKQSGAEVKKPGASVKVSCTASGFNIKDTYIHWVRQAPGQGLEWMGEIDPANDNTKYDPKFQGRVTITADTSTSTVYMELSSLRSEDTAVYYCATYYYKYDVGGFDYWGQGTLVTVSSASTKGPSVFPLAPSSKSTSGGTAALGCLVKDYFPEPVTVSWNSGALTSGVHTFPAVLQSSGLYSLSSVVTVPSSSLGTQTYICNVNHKPSNTKVDKRVEPKSCDKTHTCPPCPAPELLGGPSVFLFPPKPKDTLMISRTPEVTCVVVDVSHEDPEVKFNWYVDGVEVHNAKTKPREEQYASTYRVVSVLTVLHQDWLNGKEYKCKVSNKALPAPIEKTISKAKGQPREPQVYTLPPSREEMTKNQVSLTCLVKGFYPSDIAVEWESNGQPENNYKTTPPVLDSDGSFFLYSKLTVDKSRWQQGNVFSCSVMHEALHNHYTQKSLSLSPG

SEQ ID NO: 185 - protein, 450 aa, Artificial Sequence
  source: /note="Description of Artificial Sequence: Synthetic polypeptide"
QVQLVQSGAEVKKPGASVKVSCKASGFNIKDTYIHWVRQAPGQGLEWMGEIDPANDNTKYDPKFQGRVTITADTSSNTVYMELSSLRSEDTAVYYCATYYYKYDVGGFDYWGQGTLVTVSSASTKGPSVFPLAPSSKSTSGGTAALGCLVKDYFPEPVTVSWNSGALTSGVHTFPAVLQSSGLYSLSSVVTVPSSSLGTQTYICNVNHKPSNTKVDKRVEPKSCDKTHTCPPCPAPELLGGPSVFLFPPKPKDTLMISRTPEVTCVVVDVSHEDPEVKFNWYVDGVEVHNAKTKPREEQYASTYRVVSVLTVLHQDWLNGKEYKCKVSNKALPAPIEKTISKAKGQPREPQVYTLPPSREEMTKNQVSLTCLVKGFYPSDIAVEWESNGQPENNYKTTPPVLDSDGSFFLYSKLTVDKSRWQQGNVFSCSVMHEALHNHYTQKSLSLSPG

SEQ ID NO: 186 - protein, 450 aa, Artificial Sequence
  source: /note="Description of Artificial Sequence: Synthetic polypeptide"
QVQMKQSGAEVKKPGASVKVSCTASGFNIKDTYIHWVRQAPGQGLEWMGEIDPANDNTKYDPKFQGRVTITADTSSNTVYMELSSLRSEDTAVYYCATYYYKYDVGGFDYWGQGTLVTVSSASTKGPSVFPLAPSSKSTSGGTAALGCLVKDYFPEPVTVSWNSGALTSGVHTFPAVLQSSGLYSLSSVVTVPSSSLGTQTYICNVNHKPSNTKVDKRVEPKSCDKTHTCPPCPAPELLGGPSVFLFPPKPKDTLMISRTPEVTCVVVDVSHEDPEVKFNWYVDGVEVHNAKTKPREEQYASTYRVVSVLTVLHQDWLNGKEYKCKVSNKALPAPIEKTISKAKGQPREPQVYTLPPSREEMTKNQVSLTCLVKGFYPSDIAVEWESNGQPENNYKTTPPVLDSDGSFFLYSKLTVDKSRWQQGNVFSCSVMHEALHNHYTQKSLSLSPG

SEQ ID NO: 187 - protein, 215 aa, Artificial Sequence
  source: /note="Description of Artificial Sequence: Synthetic polypeptide"
EIVLTQSPGTLSLSPGERATLSCSVSSSISSSNLHWYQQKPGQAPRLLIYGTSNLASGIPDRFSGSGSGTDFTLTISRLEPEDFAVYYCQQWSSYPFTFGQGTKVEIKRTVAAPSVFIFPPSDEQLKSGTASVVCLLNNFYPREAKVQWKVDNALQSGNSQESVTEQDSKDSTYSLSSTLTLSKADYEKHKVYACEVTHQGLSSPVTKSFNRGEC

SEQ ID NO: 188 - protein, 215 aa, Artificial Sequence
  source: /note="Description of Artificial Sequence: Synthetic polypeptide"
EIVLTQSPGTLSLSPGERATLSCSVSSSISSSNLHWYQQKPGQAPRLLIYGTSNLASGIPDRFSGSGSGTSYTLTISRLEPEDFAVYYCQQWSSYPFTFGQGTKVEIKRTVAAPSVFIFPPSDEQLKSGTASVVCLLNNFYPREAKVQWKVDNALQSGNSQESVTEQDSKDSTYSLSSTLTLSKADYEKHKVYACEVTHQGLSSPVTKSFNRGEC

SEQ ID NO: 189 - protein, 215 aa, Artificial Sequence
  source: /note="Description of Artificial Sequence: Synthetic polypeptide"
EILLTQSPGTLSLSPGERATLSCSVSSSISSSNLHWFQQKPGQAPRLLIYGTSNLASGIPDRFSGSGSGTSYTLTISRLEPEDFAVYYCQQWSSYPFTFGQGTKVEIKRTVAAPSVFIFPPSDEQLKSGTASVVCLLNNFYPREAKVQWKVDNALQSGNSQESVTEQDSKDSTYSLSSTLTLSKADYEKHKVYACEVTHQGLSSPVTKSFNRGEC

SEQ ID NO: 190 - protein, 215 aa, Artificial Sequence
  source: /note="Description of Artificial Sequence: Synthetic polypeptide"
EILLTQSPGTLSLSPGERATLSCSVSSSISSSNLHWFQQKPGQAPRLWIYGTSNLASGVPDRFSGSGSGTSYTLTISRLEPEDFAVYYCQQWSSYPFTFGQGTKVEIKRTVAAPSVFIFPPSDEQLKSGTASVVCLLNNFYPREAKVQWKVDNALQSGNSQESVTEQDSKDSTYSLSSTLTLSKADYEKHKVYACEVTHQGLSSPVTKSFNRGEC

SEQ ID NO: 191 - protein, 215 aa, Artificial Sequence
  source: /note="Description of Artificial Sequence: Synthetic polypeptide"
EILLTQSPGTLSLSPGERATLTCSVSSSISSSNLHWFQQKPGQSPRLWIYGTSNLASGVPDRFSGSGSGTSYTLTISRLEPEDFAVYYCQQWSSYPFTFGQGTKVEIKRTVAAPSVFIFPPSDEQLKSGTASVVCLLNNFYPREAKVQWKVDNALQSGNSQESVTEQDSKDSTYSLSSTLTLSKADYEKHKVYACEVTHQGLSSPVTKSFNRGEC

SEQ ID NO: 192 - protein, 329 aa, Homo sapiens
ASTKGPSVFPLAPSSKSTSGGTAALGCLVKDYFPEPVTVSWNSGALTSGVHTFPAVLQSSGLYSLSSVVTVPSSSLGTQTYICNVNHKPSNTKVDKRVEPKSCDKTHTCPPCPAPELLGGPSVFLFPPKPKDTLMISRTPEVTCVVVDVSHEDPEVKFNWYVDGVEVHNAKTKPREEQYNSTYRVVSVLTVLHQDWLNGKEYKCKVSNKALPAPIEKTISKAKGQPREPQVYTLPPSREEMTKNQVSLTCLVKGFYPSDIAVEWESNGQPENNYKTTPPVLDSDGSFFLYSKLTVDKSRWQQGNVFSCSVMHEALHNHYTQKSLSLSPG

SEQ ID NO: 193 - protein, 330 aa, Homo sapiens
ASTKGPSVFPLAPSSKSTSGGTAALGCLVKDYFPEPVTVSWNSGALTSGVHTFPAVLQSSGLYSLSSVVTVPSSSLGTQTYICNVNHKPSNTKVDKRVEPKSCDKTHTCPPCPAPELLGGPSVFLFPPKPKDTLMISRTPEVTCVVVDVSHEDPEVKFNWYVDGVEVHNAKTKPREEQYNSTYRVVSVLTVLHQDWLNGKEYKCKVSNKALPAPIEKTISKAKGQPREPQVYTLPPSREEMTKNQVSLTCLVKGFYPSDIAVEWESNGQPENNYKTTPPVLDSDGSFFLYSKLTVDKSRWQQGNVFSCSVMHEALHNHYTQKSLSLSPGK

SEQ ID NO: 194 - protein, 329 aa, Artificial Sequence
  source: /note="Description of Artificial Sequence: Synthetic polypeptide"
ASTKGPSVFPLAPSSKSTSGGTAALGCLVKDYFPEPVTVSWNSGALTSGVHTFPAVLQSSGLYSLSSVVTVPSSSLGTQTYICNVNHKPSNTKVDKRVEPKSCDKTHTCPPCPAPELLGGPSVFLFPPKPKDTLMISRTPEVTCVVVDVSHEDPEVKFNWYVDGVEVHNAKTKPREEQYASTYRVVSVLTVLHQDWLNGKEYKCKVSNKALPAPIEKTISKAKGQPREPQVYTLPPSREEMTKNQVSLTCLVKGFYPSDIAVEWESNGQPENNYKTTPPVLDSDGSFFLYSKLTVDKSRWQQGNVFSCSVMHEALHNHYTQKSLSLSPG

SEQ ID NO: 195 - protein, 330 aa, Artificial Sequence
  source: /note="Description of Artificial Sequence: Synthetic polypeptide"
ASTKGPSVFPLAPSSKSTSGGTAALGCLVKDYFPEPVTVSWNSGALTSGVHTFPAVLQSSGLYSLSSVVTVPSSSLGTQTYICNVNHKPSNTKVDKRVEPKSCDKTHTCPPCPAPELLGGPSVFLFPPKPKDTLMISRTPEVTCVVVDVSHEDPEVKFNWYVDGVEVHNAKTKPREEQYASTYRVVSVLTVLHQDWLNGKEYKCKVSNKALPAPIEKTISKAKGQPREPQVYTLPPSREEMTKNQVSLTCLVKGFYPSDIAVEWESNGQPENNYKTTPPVLDSDGSFFLYSKLTVDKSRWQQGNVFSCSVMHEALHNHYTQKSLSLSPGK

SEQ ID NO: 196 - protein, 326 aa, Artificial Sequence
  source: /note="Description of Artificial Sequence: Synthetic polypeptide"
ASTKGPSVFPLAPCSRSTSESTAALGCLVKDYFPEPVTVSWNSGALTSGVHTFPAVLQSSGLYSLSSVVTVPSSSLGTKTYTCNVDHKPSNTKVDKRVESKYGPPCPPCPAPEFLGGPSVFLFPPKPKDTLMISRTPEVTCVVVDVSQEDPEVQFNWYVDGVEVHNAKTKPREEQFNSTYRVVSVLTVLHQDWLNGKEYKCKVSNKGLPSSIEKTISKAKGQPREPQVYTLPPSQEEMTKNQVSLTCLVKGFYPSDIAVEWESNGQPENNYKTTPPVLDSDGSFFLYSRLTVDKSRWQEGNVFSCSVMHEALHNHYTQKSLSLSLG

SEQ ID NO: 197 - protein, 327 aa, Artificial Sequence
  source: /note="Description of Artificial Sequence: Synthetic polypeptide"
ASTKGPSVFPLAPCSRSTSESTAALGCLVKDYFPEPVTVSWNSGALTSGVHTFPAVLQSSGLYSLSSVVTVPSSSLGTKTYTCNVDHKPSNTKVDKRVESKYGPPCPPCPAPEFLGGPSVFLFPPKPKDTLMISRTPEVTCVVVDVSQEDPEVQFNWYVDGVEVHNAKTKPREEQFNSTYRVVSVLTVLHQDWLNGKEYKCKVSNKGLPSSIEKTISKAKGQPREPQVYTLPPSQEEMTKNQVSLTCLVKGFYPSDIAVEWESNGQPENNYKTTPPVLDSDGSFFLYSRLTVDKSRWQEGNVFSCSVMHEALHNHYTQKSLSLSLGK

SEQ ID NO: 198 - protein, 107 aa, Homo sapiens [sequence omitted]

SEQ ID NO: 199 - protein, 30 aa, Homo sapiens
GPPAAAPGHPLAPGPHPAAPSSWGPRPRRY

SEQ ID NO: 200 - protein, 17 aa, Homo sapiens
AEYFQHWGQGTLVTVSS

SEQ ID NO: 201 - protein, 12 aa, Homo sapiens
WTFGQGTKVEIK

SEQ ID NO: 202 - protein, 449 aa, Artificial Sequence
  source: /note="Description of Artificial Sequence: Synthetic polypeptide"
EVQLLESGGGLVQPGGSLRLSCAASGFTFSSYIMMWVRQAPGKGLEWVSSIYPSGGITFYADTVKGRFTISRDNSKNTLYLQMNSLRAEDTAVYYCARIKLGTVTTVDYWGQGTLVTVSSASTKGPSVFPLAPSSKSTSGGTAALGCLVKDYFPEPVTVSWNSGALTSGVHTFPAVLQSSGLYSLSSVVTVPSSSLGTQTYICNVNHKPSNTKVDKRVEPKSCDKTHTCPPCPAPELLGGPSVFLFPPKPKDTLMISRTPEVTCVVVDVSHEDPEVKFNWYVDGVEVHNAKTKPREEQYNSTYRVVSVLTVLHQDWLNGKEYKCKVSNKALPAPIEKTISKAKGQPREPQVYTLPPSREEMTKNQVSLTCLVKGFYPSDIAVEWESNGQPENNYKTTPPVLDSDGSFFLYSKLTVDKSRWQQGNVFSCSVMHEALHNHYTQKSLSLSPG

SEQ ID NO: 203 - protein, 215 aa, Artificial Sequence
  source: /note="Description of Artificial Sequence: Synthetic polypeptide"
QSALTQPASVSGSPGQSITISCTGTSSDVGGYNYVSWYQQHPGKAPKLMIYDVSNRPSGVSNRFSGSKSGNTASLTISGLQAEDEADYYCSSYTSSSTRVFGTGTKVTVLQPKANPTVTLFPPSSEELQANKATLVCLISDFYPGAVTVAWKADGSPVKAGVETTKPSKQSNNKYAASSYLSLTPEQWKSHRSYSCQVTHEGSTVEKTVAPTECS

SEQ ID NO: 204 - protein, 450 aa, Artificial Sequence
  source: /note="Description of Artificial Sequence: Synthetic polypeptide"
EVQLVESGGGLVQPGGSLRLSCAASGFTFSRYWMSWVRQAPGKGLEWVANIKQDGSEKYYVDSVKGRFTISRDNAKNSLYLQMNSLRAEDTAVYYCAREGGWFGELAFDYWGQGTLVTVSSASTKGPSVFPLAPSSKSTSGGTAALGCLVKDYFPEPVTVSWNSGALTSGVHTFPAVLQSSGLYSLSSVVTVPSSSLGTQTYICNVNHKPSNTKVDKRVEPKSCDKTHTCPPCPAPELLGGPSVFLFPPKPKDTLMISRTPEVTCVVVDVSHEDPEVKFNWYVDGVEVHNAKTKPREEQYNSTYRVVSVLTVLHQDWLNGKEYKCKVSNKALPAPIEKTISKAKGQPREPQVYTLPPSREEMTKNQVSLTCLVKGFYPSDIAVEWESNGQPENNYKTTPPVLDSDGSFFLYSKLTVDKSRWQQGNVFSCSVMHEALHNHYTQKSLSLSPG

SEQ ID NO: 205 - protein, 215 aa, Artificial Sequence
  source: /note="Description of Artificial Sequence: Synthetic polypeptide"
EIVLTQSPGTLSLSPGERATLSCRASQRVSSSYLAWYQQKPGQAPRLLIYDASSRATGIPDRFSGSGSGTDFTLTISRLEPEDFAVYYCQQYGSLPWTFGQGTKVEIKRTVAAPSVFIFPPSDEQLKSGTASVVCLLNNFYPREAKVQWKVDNALQSGNSQESVTEQDSKDSTYSLSSTLTLSKADYEKHKVYACEVTHQGLSSPVTKSFNRGEC

SEQ ID NO: 206 - protein, 447 aa, Artificial Sequence
  source: /note="Description of Artificial Sequence: Synthetic polypeptide"
EVQLVESGGGLVQPGGSLRLSCAASGFTFSDSWIHWVRQAPGKGLEWVAWISPYGGSTYYADSVKGRFTISADTSKNTAYLQMNSLRAEDTAVYYCARRHWPGGFDYWGQGTLVTVSSASTKGPSVFPLAPSSKSTSGGTAALGCLVKDYFPEPVTVSWNSGALTSGVHTFPAVLQSSGLYSLSSVVTVPSSSLGTQTYICNVNHKPSNTKVDKRVEPKSCDKTHTCPPCPAPELLGGPSVFLFPPKPKDTLMISRTPEVTCVVVDVSHEDPEVKFNWYVDGVEVHNAKTKPREEQYNSTYRVVSVLTVLHQDWLNGKEYKCKVSNKALPAPIEKTISKAKGQPREPQVYTLPPSREEMTKNQVSLTCLVKGFYPSDIAVEWESNGQPENNYKTTPPVLDSDGSFFLYSKLTVDKSRWQQGNVFSCSVMHEALHNHYTQKSLSLSPG

SEQ ID NO: 207 - protein, 214 aa, Artificial Sequence
  source: /note="Description of Artificial Sequence: Synthetic polypeptide"
DIQMTQSPSSLSASVGDRVTITCRASQDVSTAVAWYQQKPGKAPKLLIYSASFLYSGVPSRFSGSGSGTDFTLTISSLQPEDFATYYCQQYLYHPATFGQGTKVEIKRTVAAPSVFIFPPSDEQLKSGTASVVCLLNNFYPREAKVQWKVDNALQSGNSQESVTEQDSKDSTYSLSSTLTLSKADYEKHKVYACEVTHQGLSSPVTKSFNRGEC

SEQ ID NO: 208 - protein, 329 aa, Homo sapiens
ASTKGPSVFPLAPSSKSTSGGTAALGCLVKDYFPEPVTVSWNSGALTSGVHTFPAVLQSSGLYSLSSVVTVPSSSLGTQTYICNVNHKPSNTKVDKKVEPKSCDKTHTCPPCPAPELLGGPSVFLFPPKPKDTLMISRTPEVTCVVVDVSHEDPEVKFNWYVDGVEVHNAKTKPREEQYNSTYRVVSVLTVLHQDWLNGKEYKCKVSNKALPAPIEKTISKAKGQPREPQVYTLPPSRDELTKNQVSLTCLVKGFYPSDIAVEWESNGQPENNYKTTPPVLDSDGSFFLYSKLTVDKSRWQQGNVFSCSVMHEALHNHYTQKSLSLSPG

SEQ ID NO: 209 - protein, 330 aa, Homo sapiens [sequence omitted]

SEQ ID NO: 210 - protein, 503 aa, Homo sapiens
LQPGAEVPVVWAQEGAPAQLPCSPTIPLQDLSLLRRAGVTWQHQPDSGPPAAAPGHPLAPGPHPAAPSSWGPRPRRYTVLSVGPGGLRSGRLPLQPRVQLDERGRQRGDFSLWLRPARRADAGEYRAAVHLRDRALSCRLRLRLGQASMTASPPGSLRASDWVILNCSFSRPDRPASVHWFRNRGQGRVPVRESPHHHLAESFLFLPQVSPMDSGPWGCILTYRDGFNVSIMYNLTVLGLEPPTPLTVYAGAGSRVGLPCRLPAGVGTRSFLTAKWTPPGGGPDLLVTGDNGDFTLRLEDVSQAQAGTYTCHIHLQEQQLNATVTLAIITVTPKSFGSPGSLGKLLCEVTPVSGQERFVWSSLDTPSQRSFSGPWLEAQEAQLLSQPWQCQLYQGERLLGAAVYFTELSSPGAQRSGRAPGALPAGHLLLFLILGVLSLLLLVTGAFGFHLWRRQWRPRRFSALEQGIHPPQAQSKIEELEQEPEPEPEPEPEPEPEPEPEQL

SEQ ID NO: 211 - protein, 7 aa, Homo sapiens
PTIPLQD

SEQ ID NO: 212 - protein, 8 aa, Homo sapiens
SPTIPLQD

SEQ ID NO: 213 - protein, 9 aa, Homo sapiens
SPTIPLQDL

SEQ ID NO: 214 - protein, 10 aa, Homo sapiens
SPTIPLQDLS

SEQ ID NO: 215 - protein, 11 aa, Homo sapiens
SPTIPLQDLSL

SEQ ID NO: 216 - protein, 12 aa, Homo sapiens
SPTIPLQDLSLL

SEQ ID NO: 217 - protein, 428 aa, Homo sapiens
LQPGAEVPVVWAQEGAPAQLPCSPTIPLQDLSLLRRAGVTWQHQPDSGPPAAAPGHPLAPGPHPAAPSSWGPRPRRYTVLSVGPGGLRSGRLPLQPRVQLDERGRQRGDFSLWLRPARRADAGEYRAAVHLRDRALSCRLRLRLGQASMTASPPGSLRASDWVILNCSFSRPDRPASVHWFRNRGQGRVPVRESPHHHLAESFLFLPQVSPMDSGPWGCILTYRDGFNVSIMYNLTVLGLEPPTPLTVYAGAGSRVGLPCRLPAGVGTRSFLTAKWTPPGGGPDLLVTGDNGDFTLRLEDVSQAQAGTYTCHIHLQEQQLNATVTLAIITVTPKSFGSPGSLGKLLCEVTPVSGQERFVWSSLDTPSQRSFSGPWLEAQEAQLLSQPWQCQLYQGERLLGAAVYFTELSSPGAQRSGRAPGALPAGHL

SEQ ID NO: 218 - protein, 121 aa, Artificial Sequence; identical to SEQ ID NO: 65
  source: /note="Description of Artificial Sequence: Synthetic polypeptide"
  VARIANT (4)..(4): /replace="L"
  VARIANT (5)..(5): /replace="K"
  VARIANT (12)..(12): /replace="V"
  VARIANT (23)..(23): /replace="T"
  VARIANT (48)..(48): /replace="I"
  VARIANT (70)..(70): /replace="M"
  VARIANT (72)..(72): /replace="R"
  VARIANT (76)..(76): /replace="S"
  VARIANT (77)..(77): /replace="N"
  VARIANT (81)..(81): /replace="L"
  VARIANT (82)..(82): /replace="Q"
  VARIANT (98)..(98): /replace="R"
  VARIANT (102)..(102): /replace="R"
  VARIANT (104)..(104): /replace="E"
  MISC_FEATURE (1)..(121): /note="Variant residues given in the sequence have no preference with respect to those in the annotations for variant positions"

SEQ ID NO: 219 - protein, 107 aa, Homo sapiens
GTVAAPSVFIFPPSDEQLKSGTASVVCLLNNFYPREAKVQWKVDNALQSGNSQESVTEQDSKDSTYSLSSTLTLSKADYEKHKVYACEVTHQGLSSPVTKSFNRGEC

SEQ ID NO: 220 - protein, 121 aa, Artificial Sequence; identical to SEQ ID NO: 65
  source: /note="Description of Artificial Sequence: Synthetic polypeptide"
  VARIANT (1)..(1): /replace="pE (pyroglutamate)"
  MISC_FEATURE (1)..(121): /note="Variant residues given in the sequence have no preference with respect to those in the annotations for variant positions"

SEQ ID NO: 221 - protein, 108 aa, Artificial Sequence; identical to SEQ ID NO: 73
  source: /note="Description of Artificial Sequence: Synthetic polypeptide"
  VARIANT (1)..(1): /replace="pE (pyroglutamate)"
  MISC_FEATURE (1)..(108): /note="Variant residues given in the sequence have no preference with respect to those in the annotations for variant positions"

SEQ ID NO: 222 - protein, 121 aa, Artificial Sequence; identical to SEQ ID NO: 65
  source: /note="Description of Artificial Sequence: Synthetic polypeptide"
  VARIANT (1)..(1): /replace="pE (pyroglutamate)"
  VARIANT (4)..(4): /replace="L"
  VARIANT (5)..(5): /replace="K"
  VARIANT (12)..(12): /replace="V"
  VARIANT (48)..(48): /replace="I"
  VARIANT (70)..(70): /replace="M"
  VARIANT (72)..(72): /replace="R"
  VARIANT (76)..(76): /replace="S"
  VARIANT (77)..(77): /replace="N"
  VARIANT (81)..(81): /replace="L"
  VARIANT (82)..(82): /replace="Q"
  VARIANT (98)..(98): /replace="R"
  VARIANT (102)..(102): /replace="R"
  VARIANT (104)..(104): /replace="E"
  MISC_FEATURE (1)..(121): /note="Variant residues given in the sequence have no preference with respect to those in the annotations for variant positions"

SEQ ID NO: 223 - protein, 121 aa, Artificial Sequence; identical to SEQ ID NO: 65
  source: /note="Description of Artificial Sequence: Synthetic polypeptide"
  VARIANT (1)..(1): /replace="pE (pyroglutamate)"
  VARIANT (4)..(4): /replace="L"
  VARIANT (5)..(5): /replace="K"
  VARIANT (12)..(12): /replace="V"
  VARIANT (23)..(23): /replace="T"
  VARIANT (48)..(48): /replace="I"
  VARIANT (70)..(70): /replace="M"
  VARIANT (72)..(72): /replace="R"
  VARIANT (76)..(76): /replace="S"
  VARIANT (77)..(77): /replace="N"
  VARIANT (81)..(81): /replace="L"
  VARIANT (82)..(82): /replace="Q"
  VARIANT (98)..(98): /replace="R"
  VARIANT (102)..(102): /replace="R"
  VARIANT (104)..(104): /replace="E"
  MISC_FEATURE (1)..(121): /note="Variant residues given in the sequence have no preference with respect to those in the annotations for variant positions"

SEQ ID NO: 224 - protein, 108 aa, Artificial Sequence; identical to SEQ ID NO: 73
  source: /note="Description of Artificial Sequence: Synthetic polypeptide"
  VARIANT (1)..(1): /replace="pE (pyroglutamate)"
  VARIANT (3)..(3): /replace="L"
  VARIANT (22)..(22): /replace="T"
  VARIANT (37)..(37): /replace="F"
  VARIANT (44)..(44): /replace="S"
  VARIANT (48)..(48): /replace="W"
  VARIANT (59)..(59): /replace="V"
  VARIANT (71)..(71): /replace="S"
  VARIANT (72)..(72): /replace="Y"
  MISC_FEATURE (1)..(108): /note="Variant residues given in the sequence have no preference with respect to those in the annotations for variant positions"

SEQ ID NO: 225 - protein, 450 aa, Artificial Sequence; identical to SEQ ID NO: 168
  source: /note="Description of Artificial Sequence: Synthetic polypeptide"
  VARIANT (1)..(1): /replace="pE (pyroglutamate)"
  MISC_FEATURE (1)..(450): /note="Variant residues given in the sequence have no preference with respect to those in the annotations for variant positions"

SEQ ID NO: 226 - protein, 450 aa, Artificial Sequence; identical to SEQ ID NO: 169
  source: /note="Description of Artificial Sequence: Synthetic polypeptide"
  VARIANT (1)..(1): /replace="pE (pyroglutamate)"
  MISC_FEATURE (1)..(450): /note="Variant residues given in the sequence have no preference with respect to those in the annotations for variant positions"

SEQ ID NO: 227 - protein, 447 aa, Artificial Sequence; identical to SEQ ID NO: 170
  source: /note="Description of Artificial Sequence: Synthetic polypeptide"
  VARIANT (1)..(1): /replace="pE (pyroglutamate)"
  MISC_FEATURE (1)..(447): /note="Variant residues given in the sequence have no preference with respect to those in the annotations for variant positions"

SEQ ID NO: 228 - protein, 215 aa, Artificial Sequence; identical to SEQ ID NO: 187
  source: /note="Description of Artificial Sequence: Synthetic polypeptide"
  VARIANT (1)..(1): /replace="pE (pyroglutamate)"
  MISC_FEATURE (1)..(215): /note="Variant residues given in the sequence have no preference with respect to those in the annotations for variant positions"